European Patent Application EP 4 636 095 A1, published October 22, 2025. Title: Preeclampsia biomarker and use thereof. Applicant: BGI GENOMICS CO., LTD. Application EP. The sequence listing filed with the application follows.

SEQUENCE LISTING (18 sequences)

SEQ ID NO: 1 - DNA, 17196 bp, Homo sapiens
  source 1..17196: mol_type = other DNA
ctagcttttctcttctgtcaaccccacacgcctttggcacaatgaagtgggtaacctttatttcccttctttttctctttagctcggcttattccaggggtgtgtttcgtcgagatgcacgtaagaaatccatttttctattgttcaacttttattctattttcccagtaaaataaagttttagtaaactctgcatctttaaagaattattttggcatttatttctaaaatggcatagtattttgtatttgtgaagtcttacaaggttatcttattaataaaattcaaacatcctaggtaaaaaaaaaaaaaggtcagaattgtttagtgactgtaattttcttttgcgcactaaggaaagtgcaaagtaacttagagtgactgaaacttcacagaatagggttgaagattgaattcataactatcccaaagacctatccattgcactatgctttatttaaaaaccacaaaacctgtgctgttgatctcataaatagaacttgtatttatatttattttcattttagtctgtcttcttggttgctgttgatagacactaaaagagtattagatattatctaagtttgaatataaggctataaatatttaataatttttaaaatagtattcttggtaattgaattattcttctgtttaaaggcagaagaaataattgaacatcatcctgagtttttctgtaggaatcagagcccaatattttgaaacaaatgcataatctaagtcaaatggaaagaaatataaaaagtaacattattacttcttgttttcttcagtatttaacaatccttttttttcttcccttgcccagacaagagtgaggttgctcatcggtttaaagatttgggagaagaaaatttcaaagccttgtaagttaaaatattgatgaatcaaatttaatgtttctaatagtgttgtttattattctaaagtgcttatatttccttgtcatcagggttcagattctaaaacagtgctgcctcgtagagttttctgcgttgaggaagatattctgtatctgggctatccaataaggtagtcactggtcacatggctattgagtacttcaaatatgacaagtgcaactgagaaacaaaaacttaaattgtatttaattgtagttaatttgaatgtatatagtcacatgtggctaatggctactgtattggacagtacagctctggaacttgcttggtggaaaggactttaatataggtttcctttggtggcttacccactaaatcttctttacatagcaagcattcctgtgcttagttgggaatatttaatttttttttttttttaagacagggtctcgctctgtcgcccaggctggagtgcagtggcgcaatctcggctcactgcaaactccgcctcccgggttcacgccattctcctgcctcagcctcccgagtagctgggactacaggcgcccgccatcacgcccggctaatcttttgtatttttagtagagatggggtttcaccgtgtgccaggatggtctcaatctcctgacatcgtgatctgcccacctcggcctcccaaagtgctgggattacaggagtgagccaccgcgcccggcctatttaaatgttttttaatctagtaaaaaatgagaaaattgtttttttaaaagtctacctaatcctacaggctaattaaagacgtgtgtggggatcaggtgcggtggttcacacctgtaatcccagcactttggaaggctgatgcaggaggattgcttgagcccaggagttcaagaccagcctgggcaagtctctttaaaaaaaacaaaacaaacaaacaaaaaaattaggcatggtggcacatgcctgtagtcctagctacttaggaggctgacgtaggaggatcgtttggacctgagaggtcaaggctacagtgagccatgattgtgccactgcactccagcctgggtgacagagtgagactctgtctcaaaaaagaaaaaggaaatctgtggggtttgttttagttttaagtaattctaaggactttaaaaatgcctagtcttgacaattagatctatttggcatacaatttgcttgcttaatctatgtgtgtgcatagatctactgacacacgcatacatataaacattagggaactaccattctctttgcgtaggaagccacatatgcctatctaggcctcagatcatacctgatatgaataggctttctggataatggtgaagaagatgtataaaagatagaacctatacccatacatgatttgttctctagcgtagcaacctgttacatattaaagttttattatactacatttttctacatcctttgtttcagggtgttgattgcctttgctcagtatcttcagcagtgtccatttgaagatcatgtaaaattagtgaatgaagtaactgaatttgcaaaaacatgtgttgctgatgagtcagctgaaaattgtgacaaatcacttgtaagtacattctaattgtggagattctttcttctgtttgaagtaatcccaagcatttcaaaggaattttttttaagttttctcaattattattaagtgtcctgatttgtaagaaacactaaaaagttgctcatagactgataagccattgtttcttttgtgatagagatgctttagctatgtccacagttttaaaatcatttctttattgagaccaaacacaacagtcatggtgtatttaaatggcaatttgtcatttataaacacctctttttaaaatttgaggtttggtttctttttgtagaggctaatagggatatgatagcatgtatttatttatttatttatcttattttattatagtaagaacccttaacatgagatctaccctgttatatttttaagtgtacaatccattattgttaactacgggtacactgttgtatagcttactcatcttgctgtattaaaactttgtgcccattgattagtaacccctcgtttcgtcctcccccagccactggcaaccagcattatactctttgattctatgagtttgactactttagctaccttatataagtggtattatgtactgtttatctttttatgactgacttatttcccttagcatagtgcattcaaagtccaaccatgttgttgcctattgcagaatttccttcttttcaaggctgaataatattccagtgcatgtgtgtaccacattttctttatccattaatttgttgattgatagacatttaggttggttttctacatcttgactatcatgaatagtgttgcaatgaacacaggagagctactatctcttagagatgatatcatggtttttatcatcagaaaacacccactgatttctatgctaattttgttacctgggtggaataatagtacagctatatattcctcattttagatatctttgtatttctacatacaataaaaaagcagagtacttagtcatgttgaagaactttaaacttttagtatttccagatcaatcttcaaaacaaggacaggtttatctttctctcaccactcaatctatatatacctcttgtgggcaaggccagtttttatcactggagcctttcccctttttattatgtacctctccctcacagcagagtcaggactttaactttacacaatactatggctctacatatgaaatcttaaaaatacataaaaattaataaattctgtctagagtagtatattttccctggggttacagttactttcataataaaaattagagataaggaaaggactcatttattggaaagtgattttaggtaacatttctggaagaaaaatgtctatatcttaatagtcacttaatatatgatggattgtgttactcctcagttttcaatggcatatactaaaacatggccctctaaaaagggggcaaatgaaatgagaaactctctgaatgtttttctcccctaggtgaattcacctgctgcttagaagcttattttctcttgatttctgttataatgattgctcttaccctttagttttaagtttcaaaataggagtcatataactttccttaaagctattgactgtctttttgtcctgttttattcaccatgagttatagtgtgacagttaattcttatgaaaattatatagagatggttaaatcatcagaaactgtaaacctcgattgggaggggaagcggatttttaaatgatttcctgaccaagcttaaccagtatattaaatcctttgtactgttctttggctataaagaaaaaaggtactgtccagcaactgaaacctgctttcttccatttagcataccctttttggagacaaattatgcacagttgcaactcttcgtgaaacctatggtgaaatggctgactgctgtgcaaaacaagaacctgagagaaatgaatgcttcttgcaacacaaagatgacaacccaaacctcccccgattggtgagaccagaggttgatgtgatgtgcactgcttttcatgacaatgaagagacatttttgaaaaagtaagtaatcagatgtttatagttcaaaattaaaaagcatggagtaactccataggccaacactctataaaaattaccataacaaaaatattttcaacattaagacttggaagttttgttatgatgattttttaaagaagtagtatttgataccacaaaattctacacagcaaaaaatatgatcaaagatattttgaagtttattgaaacaggatacaatctttctgaaaaatttaagatagacaaattatttaatgtattacgaagatatgtatatatggttgttataattgatttcgttttagtcagcaacattatattgccaaaatttaaccatttatgcacacacacacacacacacacacacttaacccttttttccacatacttaaagaatgacagagacaagaccatcatgtgcaaattgagcttaattggttaattagatatctttggaatttggaggttctggggagaatgtcgattacaattatttctgtaatattgtctgctatagaaaagtgactgtttttctttttcaaaatttagatacttatatgaaattgccagaagacatccttacttttatgccccggaactccttttctttgctaaaaggtataaagctgcttttacagaatgttgccaagctgctgataaagctgcctgcctgttgccaaaggtattatgcaaaagaatagaaaaaaagagttcattatccaacctgattttgtccattttgtggctagatttagggaacctgagtgtctgatacaaactttccgacatggtcaaaaaagccttccttttatctgtcttgaaaatctttcatctttgaaggcctacactctcgtttcttcttttaagatttgccaatgatgatctgtcagaggtaatcactgtgcatgtgtttaaagatttcaccactttttatggtggtgatcactatagtgaaatactgaaacttgtttgtcaaattgcacagcaaggggccacagttcttgtttatcttttcatgataatttttagtagggagggaattcaaagtagagaattttactgcatctagatgcctgagttcatgcattcattccataaatatatattatggaatgctttattttcttttctgaggagtttactgatgttggtggaggagagactgaaatgaattatacacaaaatttaaaaattagcaaaattgcagcccctgggatattagcgtactctttctctgacttttctcccacttttaaggctctttttcctggcaatgtttccagttggtttctaactacatagggaattccgctgtgaccagaatgatcgaatgatctttccttttcttagagagcaaaatcattattcgctaaagggagtacttgggaatttaggcataaattatgccttcaaaatttaatttggcacagtctcatctgagcttatggaggggtgtttcatgtagaatttttcttctaattttcatcaaattattcctttttgtagctcgatgaacttcgggatgaagggaaggcttcgtctgccaaacagagactcaagtgtgccagtctccaaaaatttggagaaagagctttcaaagcatggtaaatacttttaaacatagttggcatctttataacgatgtaaatgataatgcttcagtgacaaattgtacatttttatgtattttgcaaagtgctgtcaaatacatttctttggttgtctaacaggtagaactctaatagaggtaaaaatcagaatatcaatgacaatttgacattatttttaatcttttcttttctaaatagttgaataatttagaggacgctgtcctttttgtcctaaaaaaagggacagatatttaagttctatttatttataaaatcttggactcttattctaatggttcattatttttatagagctgtaggcatggttctttatttaattttttaaagttatttttaatttttgtggatacagagtaggtatacatatttacggggtatatgagatattttgatataagtatacaacatatataatccctttatttaattttatcttccccccaatgatctaaaactatttgcttgtccttttatgtcttatagttaaattcagtcaccaactaagttgaagttacttcttatttttgcatagctccagctctgatcttcatctcatgtttttgcctgagcctctgttttcatattacttagttggttctgggagcatactttaatagccgagtcaagaaaaatactagctgccccgtcacccacactcctcacctgctagtcaacagcaaatcaacacaacaggaaataaaatgaaaataatagacattatgcatgctctctagaaactgtcaattgaactgtatttgctcatcattcctaccatctacaccaccaaaatcaaccaaatttatgaaaaaaaacagccccaacataaaattatacacagataaacaggctatgattggttttgggaaagaagtcacctttacctgatttaggcaactgtgaaatgactagagaatgaagaaaattagacgtttacatcttgtcatagagtttgaagatagtgctggatctttctttttataagtaagatcaataaaaactccctcattctgtagaagttatgatttcttttctaagagacctttagaagtcagaaaaaatgtgtttcaattgagaaaaaagataactggagtttgtgtagtacttcccagattataaaatgcttttgtatgtattatctaatttaatcctcaaaacttcttcaatttagcatgttgtcatgacactgcagaggctgaagctcagagaggctgagccctctgctaacaagtcctactgctaacaagtgataaagccagagctggaagtcacatctggactccaaacctgatgcttctcagcctgttgccccttttagagttcctttttaatttctgcttttatgacttgctagatttctacctaccacacacactcttaaatggataattctgccctaaggataagtgattaccatttggttcagaactagaactaatgaattttaaaaattatttctgtatgtccattttgaattttcttatgagaaatagtatttgcctagtgttttcatataaaatatcgcatgataataccattttgattggcgattttctttttagggcagtagctcgcctgagccagagatttcccaaagctgagtttgcagaagtttccaagttagtgacagatcttaccaaagtccacacggaatgctgccatggagatctgcttgaatgtgctgatgacagggtaaagagtcgtcgatatgctttttggtagcttgcatgctcaagttggtagaatggatgcgtttggtatcattggtgatagctgacagtgggttgagattgtcttctgtgctttcgtctgtcctatcttcaatctttccctgcctatggtggtggtacctttctgtttttaacctggctataaattaccagataaacccattcactgatttgtaactcctttcagtcatgctctaactgtaaatgaaggcttaaactgaagtagaacagttacaaggttttacttggcagaacatcttgcaaggtagatgtctaagaagatttttttttctttttttaagacagagtttcgctcttgtttcccaggctggggtgcaatggtgtgatcttggctcagcgcaacctctgcctcctgggttcaagtgattctcatgcctcagcctcccaagtagctgggattacaggcatgcgccaccacacctggctaattttgtatttttagtagaggcggggtttcaccatattgtccagactggtctcgaactcctgacctcaggtgatccacccgccttggcctcccaaagtgctgggattacaggcatgagccaccttgcccagcctaagaagattttttgagggaggtaggtggacttggagaaggtcactacttgaagagatttttggaaatgatgtatttttcttctctatattccttcccttaattaactctgtttgttagatgtgcaaatatttggaatgatatctcttttctcaaaacttataatattttctttctccctttcttcaagattaaacttatgggcaaatactagaatcctaatctctcatggcactttctggaaaatttaaggcggttattttatatatgtaagcagggcctatgactatgatcttgactcatttttcaaaaatcttctatattttatttagttatttggtttcaaaaggcctgcacttaattttgggggattatttggaaaaacagcattgagttttaatgaaaaaaacttaaatgccctaacagtagaaacataaaattaataaataactgagctgagcacctgctactgattagtctattttaattaagtgggaatgtttttgtagtcctatctacatctccaggtttaggagcaaacagagtatgttcatagaaggaatatgtgtatggtcttagaatacaatgaatatgttctgccaacttaataaaggtctgaggagaaagtgtagcaatgtcaattcgtgttgaacaatttccaccaacttacttataggcggaccttgccaagtatatctgtgaaaatcaagattcgatctccagtaaactgaaggaatgctgtgaaaaacctctgttggaaaaatcccactgcattgccgaagtggaaaatgatgagatgcctgctgacttgccttcattagctgctgattttgttgaaagtaaggatgtttgcaaaaactatgctgaggcaaaggatgtcttcctgggcatgtaagtagataagaaattattcttttatagctttggcatgacctcacaacttaggaggatagcctaggcttttctgtggagttgctacaatttccctgctgcccagaatgtttcttcatccttccctttcccaggctttaacaatttttgaaatagttaattagttgaatacattgtcataaaataatacatgttcatggcaaagctcaacattccttactccttaggggtatttctgaaaatacgtctagaaacattttgtgtatatataaattatgtatacttcagtcattcattccaagtgtatttcttgaacatctataatatatgtgtgtgactatgtattgcctgtctatctaactaatctaatctaatctagtctatctatctaatctatgcaatgatagcaaagaagtataaaaagaaatatagagtctgacaccaggtgctttatatttggtgaaaagaccagaagttcagtataatggcaatatggtaggcaactcaattacaaaataaatgtttacatattgtcagaagttgtggtgataaactgcatttttgttgttggattatgataatgcactaaataatatttcctaaaattatgtaccctacaagatttcactcatacagagaagaaagagaatattttaagaacatatctctgcccatctatttatcagaatccttttgagatgtagtttaaatcaaacaaaatgttaataaaaataacaagtatcattcatcaaagacttcatatgtgccaagcagtgtgtgctttgtgtagattatgtcatatagttctcataatccaccttccgagacagatactatttattttttgagacagagttttactcttgttgcccaggctggagtgcaatggtgccatctcggctcaccacaacctccgcctcccaggttcaagcgattctcctgcctcagcctcctgggattacaggcatgcaccaccatgcctggctaattttgtatttttagtagagatggggtttcaccatgttggtcagactggtctcaaactcctgacctctggtgatatgcctgcctcagcctcctaaagtgctgggattacaggcatgagccactgtgcccagccgacagatactattattatttccattctaccgagaaggagactaaggctctgatcatttaaataagttgcctaaggtgatgcagtgatataagtagcagagctaggaattgagccttggtaactttaactctggaccccaagtccttagctactaagctttactgcatggggtttagtcaaattaagacttttggaatatgagttacttttgagattagctttgtgatattttttgtgctcatttgtccaacaaagtctattttattttcatcttaattaggtttttgtatgaatatgcaagaaggcatcctgattactctgtcgtgctgctgctgagacttgccaagacatatgaaaccactctagagaagtgctgtgccgctgcagatcctcatgaatgctatgccaaagtggtaggtttattgttggaaaaaaatgtagttctttgactgatgattccaataatgagaaagaaaaataatgcaagaatgtaaaatgatatacagtgcaatttagatcttttcttgagatggtttcaattctggaatcttaaacatgaaagaaaaagtagccttagaatgattaacaaaatttagactagttagaatagaaagatctgaatagagcaatctctaaaaaattttgatctttttttctctttttcacaatcctgagaacaaaaaaaaattaaatttaaatgttaattagaagatatttaacttagatgtaaagtgagttaacctgattccaggattaatcaagtactagaattagtatcttatggcaaattatagaacctatccctttagaatattttcaaatctttttgaggatgtttaggaatagttttacaagaaattaagttaggagaggaaatctgttctggaggatttttagggttcccactagcatatgtaatggtttctgaactattcagaatcagagaaaactcatttttcctgctttcaagaagctactgtatgccaggcaccatgcacaaacaatgaccaacgtaaaatctctcattttggagagcctggaatctaactggaaaggtgaactaataataataatatgtacaatcatagccatcatttattaaacttttattatatgcaaggcactgtttaatttcattagcttacctggtttacagagcagctctatgagatgagtgccatctttgcccctattttagggataaggattctgaaatgtggagatggtaagtaaaattgcacaactgaagaatgagttacatgacttggctcaaatactggtcattgaactccagagcctgaatattcttaaccacttacatgatgcaagctcaccaaataaatagttcgaatgtattgtgacagagcggcattgatattcatctattcatgtggctttgagtaggaagaagaaaggatatcattctgaccagaggggtgaaaaacaacctgcatctgatcctgaggcataatactattaacacaattcttttatgtttcagttcgatgaatttaaacctcttgtggaagagcctcagaatttaatcaaacaaaattgtgagctttttgagcagcttggagagtacaaattccagaatgcgtaagtaatttttattgactgattttttttatcaatttgtaattatttaagacttaatatatgagccacctagcatagaacttttaagaatgaaaatacattgcatatttctaatcactctttgtcaagaaagataggagaggagagataaaatagttgatggggtggagaggtctatatttgaatgtagtctaaaaattgttctcttaagattggaagtatgtaggctgggagggtaaataccaaatcttggtatatcagaactgagcatgtcccttgaaggttaagaaatagttaatgggcaaatagagcatggcaatattttgtagagcagcaagtagtaggccttgaatagatgtcgctcaaaaagtaatatgtaagctgaacacaaaaatgtaacaaatgaatttagatacatatttgaatattaaattcaggttgtttgggagatgcacctagtctttgatggttaaacctttccctccatagaagagacagagacagaatggcttgctggactaatgtcccaattcaatagagtcttatctatgaaggttaaaaacaagaagagacatattatacagtagatatttattgtgtggctcatacacatggtgctcttctgattatggattttagagataataacagtgaacaagacatagtttctttcctcgagtagattaaagtcatacattgacttttaatggtgactggcattcttaatacatgattattatatattaggtaccatgtcagattaattataatactttactacttttaatttaacccttgaactatccctattgagtcagatatatttccttccattttctacttgtatctttcaagtttagcatatgctgatacatatgaagctctctccaggttttattgaaagaagaaattaataaatttattaatgtcactgaattaggcaactcactttcccaagattatgcaagtggtacaggtggaactcaaagccaagtttaactagttgttcaggagaatgttttctaccctccactaacccactactctgcagatggagataatatgatgaatggaacatagcaacatcttagttgattccggccaagtgttctctgttttatctactatgttagacagtttcttgccttgctgaaaacacatgacttctttttttcaggctattagttcgttacaccaagaaagtaccccaagtgtcaactccaactcttgtagaggtctcaagaaacctaggaaaagtgggcagcaaatgttgtaaacatcctgaagcaaaaagaatgccctgtgcagaagactatgtgagtctttaaaaaaatataataaattaataatgaaaaaattttacctttagatattgataatgctagctttcataagcagaaggaagtaatgtgtgtgtgtgcatgtttgtgtgcatgtgtgtgtgcatgcacgtgtgtgtatgtgtgatattggcagtcaaggccccgaggatgataattttttttttttttttgagacggagtctcgctttgttgtccaggctggagtgcagtggtgccatctcggctcactgcaacctccgcctcccaggttcaagccattctcctgcctcagcctcccaagtagctgggactacaggtgcatgccaccatgcctggctaattttttgtatttttagtagaaaattttcagcttcacctcttttgaatttctgctctcctgcctgttctttagctatccgtggtcctgaaccagttatgtgtgttgcatgagaaaacgccagtaagtgacagagtcaccaaatgctgcacagaatccttggtgaacaggcgaccatgcttttcagctctggaagtcgatgaaacatacgttcccaaagagtttaatgctgaaacattcaccttccatgcagatatatgcacactttctgagaaggagagacaaatcaagaaacaaacgtgaggagtatttcattactgcatgtgtttgtagtcttgatagcaagaactgtcaattcaagctagcaactttttcctgaagtagtgattatatttcttagaggaaagtattggagtgttgcccttattatgctgataagagtacccagaataaaatgaataactttttaaagacaaaatcctctgttataatattgctaaaattattcagagtaatattgtggattaaagccacaatagaataacatgttaggccatattcagtagaaaaagatgaacaattaactgataaatttgtgcacatggcaaattagttaatgggaaccataggagaatttatttctagatgtaaataattattttaagtttgccctatggtggccccacacatgagacaaacccccaagatgtgacttttgagaatgagacttggataaaaaacatgtagaaatgcaagccctgaagctcaactccctattgctatcacaggggttataattgcataaaatttagctatagaaagttgctgtcatctcttgtgggctgtaatcatcgtctaggcttaagagtaatattgcaaaacctgtcatgcccacacaaatctctccctggcattgttgtctttgcagatgtcagtgaaagagaaccagcagctcccatgagtttggatagccttattttctatagcctccccactattagctttgaagggagcaaagtttaagaaccaaatataaagtttctcatctttatagatgagaaaaattttaaataaagtccaagataattaaatttttaaggatcatttttagctctttaatagcaataaaactcaatatgacataatatggcacttccaaaatctgaataatatataattgcaatgacatacttcttttcagagatttactgaaaagaaatttgttgacactacataacgtgatgagtggtttatactgattgtttcagttggtcttcccaccaactccatgaaagtggattttattatcctcatcatgcagatgagaatattgagacttatagcggtatgcctgagccccaaagtactcagagttgcctggctccaagatttataatcttaaatgatgggactaccatccttactctctccatttttctatacgtgagtaatgttttttctgttttttttttttctttttccattcaaactcagtgcacttgttgagctcgtgaaacacaagcccaaggcaacaaaagagcaactgaaagctgttatggatgatttcgcagcttttgtagagaagtgctgcaaggctgacgataaggagacctgctttgccgaggaggtactacagttctcttcattttaatatgtccagtattcatttttgcatgtttggttaggctagggcttagggatttatatatcaaaggaggctttgtacatgtgggacagggatcttattttacaaacaattgtcttacaaaatgaataaaacagcactttgtttttatctcctgctctattgtgccatactgttaaatgtttataatgcctgttctgtttccaaatttgtgatgcttatgaatattaataggaatatttgtaaggcctgaaatattttgatcatgaaatcaaaacattaatttatttaaacatttacttgaaatgtggtggtttgtgatttagttgattttataggctagtgggagaatttacattcaaatgtctaaatcacttaaaattgccctttatggcctgacagtaacttttttttattcatttggggacaactatgtccgtgagcttccgtccagagattatagtagtaaattgtaattaaaggatatgatgcacgtgaaatcactttgcaatcatcaatagcttcataaatgttaattttgtatcctaatagtaatgctaatattttcctaacatctgtcatgtctttgtgttcagggtaaaaaacttgttgctgcaagtcaagctgccttaggcttataacatcacatttaaaagcatctcaggtaactatattttgaattttttaaaaaagtaactataatagttattattaaaatagcaaagattgaccatttccaagagccatatagaccagcaccgaccactattctaaactatttatgtatgtaaatattagcttttaaaattctcaaaatagttgctgagttgggaaccactattatttctattttgtagatgagaaaatgaagataaacatcaaagcatagattaagtaattttccaaagggtcaaaattcaaaattgaaaccaaagtttcagtgttgcccattgtcctgttctgacttatatgatgcggtacacagagccatccaagtaagtgatggctcagcagtggaatactctgggaattaggctgaaccacatgaaagagtgctttatagggcaaaaacagttgaatatcagtgatttcacatggttcaacctaatagttcaactcatcctttccattggagaatatgatggatctaccttctgtgaactttatagtgaagaatctgctattacatttccaatttgtcaacatgctgagctttaataggacttatcttcttatgacaacatttattggtgtgtccccttgcctagcccaacagaagaattcagcagccgtaagtctaggacaggcttaaattgttttcactggtgtaaattgcagaaagatgatctaagtaatttggcatttattttaataggtttgaaaaacacatgccattttacaaataagacttatatttgtccttttgtttttcagcctaccatgagaataagagaaagaaaatgaagatcaaaagcttattcatctgtttttctttttcgttggtgtaaagccaacaccctgtctaaaaaacataaatttctttaatcattttgcctcttttctctgtgcttcaattaataaaaaatggaaagaatctaatagagtggtacagcactgttatttttcaaagatgtgttgctatcctgaaaattctgtaggttctgtggaagttccagtgttctctcttattccacttcggtagaggatttctagtttcttgtgggctaattaaataaatcattaatactcttctaagttatggattataaacattcaaaataatattttgacattatgataattctgaataaaagaacaaaaacca

SEQ ID NO: 2 - DNA, 7617 bp, Homo sapiens
  source 1..7617: mol_type = other DNA
aatcctttctttcagctggagtgctcctcaggagccagccccacccttagaaaagatgttttccatgaggatcgtctgcctggtcctaagtgtggtgggcacagcatgggtatggcccttttcattttttcttcttgctttctctctggtgtttattccacaaagagcctggaggtcagagtctacctgctctatgtcctgacacactcttagctttatgaccccaggcctgggaggaaatttcctgggtgggcttgacacctcaagaatacagggtaatatgacaccaagaggaagatcttagatggatgagagtgtacaaactcacaagggaaactttagcatctgtcattcagtcttaccacattttgttttgttttgttttaaaaagggcaagaattatttgccatccttgtacctataaagccttggtgcattataatgctagttaatggaataaaacattttatggtaagatttgttttctttagttattaatttcttgctacttgtccataataagcagaacttttagtgttagtacagttttgctgaaaggttattgttgtgtttgtcaagacagaagaaaaagcaaacgaattatctttggaaatatctttgcagtatcagaagagattagttagtaaggcaatacgcttttccgcagtaatggtattcttttaaattatgaatccatctctaaaggttacatagaaacttgaaggagagaggaacattcagttaagatagtctaggtttttctactgaagcagcaattacaggagaaagagctctacagtagttttcaactttctgtctgcagtcattagtaaaaatgaaaaggtaaaatttaactgattttatagattcaaataattttccttttaggatggattctttaaaactcctaatatttatcaaatgcttatttaagtgtcacacacagttaagaaatttgtacaccttgtctcctttaattctcataacaactccataaaatgggtcctaggatttccatttgaagataagaaacctgaagcttgccgaagccctgtgtctgctctccttaatctctgtgagagtgccatctcttcctggggacttgtaggcatgccactgtctcctcttctggctaacattgctgttgctctcttttgtgtatgtgaatgaatctttaaagactgcagatagtggtgaaggtgactttctagctgaaggaggaggcgtgcgtggcccaagggttgtggaaagacatcaatctgcctgcaaagattcagactggcccttctgctctgatgaagactgggtaagcagtcagcgggggaagcaggagattccttccctctgatgctagaggggctcacaggctgacctgattggtcccagaaacttttttaaatagaaaataattgaatagttacctacatagcaaataaagaaaaggaacctactcccaagagcactgtttatttacctccccaactctggatcattagtgggtgaacagacaggatttcagttgcatgctcaggcaaaaccaggctcctgagtattgtggcctcaatttcctggcacctaatttatggctaagtggaccctcattccagagtttctctgcgacctctaactagtcctcttacctacttttaagccaacttatctggaagagatagggtaggaagaaatgggggctgcatggaaacatgcaaaattattctgaatctgagagatagatccttactgtaattttctcccttcactttcagaactacaaatgcccttctggctgcaggatgaaagggttgattgatgaagtcaatcaagattttacaaacagaataaataagctcaaaaattcactatttgaatatcagaagaacaataaggattctcattcgttgaccactaatataatggaaattttgagaggcgatttttcctcagccaatagtaagtattacatatttactgctttgactttataacagaaacaacaaaaatcctaaataaatatgatatccgcttatatctatgacaatttcatcccaaagtacttagtgtagaaacacataccttcataatatccctgaaaattttaagagggagcttttgttttcgttattttttcaaagtaaaagatgttaactgagattgtttaaggtcacaaaataagtcagaattttggattaaaaacaagaatttaaatgtgttcttttcaacagtatatactgaaagtaggatgggtcagactctttgagttgatatttttgtttctgctttgtaaaggtgaaaactgagaggtcaaggaacttgttcaaagacacagagctgggaattcaactcccagactccactgagctgattaggtagatttttaaatttaaaatatagggtcaagctacgtcattctcacagtctactcattagggttaggaaacattgcattcactctgggcatggacagcgagtctagggagtcctcagtttctcaagttttgctttgcctttttacaccttcacaaacacttgacatttaaaatcagtgatgcaacactagctggcaagtgagtgatcctgttgacccaaaacagcttaggaaccatttcaaatctatagattaaaaagaaaagctcatcagtaagaaaatccaatatgttcaagtcccttgattaaggatgttataaaataattgaaatgcaatcaaaccaactattttaactccaaattacacctttaaaattccaaagaaagttcttcttctatatttctttgggattactaattgctattaggacatcttaactggcattcatggaaggctgcagggcataacattatccaaaagtcaaatgccccataggttttgaactcacagattaaactgtaaccaaaataaaattaggcatatttacaagctagtttctttctttcttttttctctttctttctttctttctttctttctttctttctttctttctttctttctttctttctccttccttcctttcttcctttcttttttgctggcaattacagacaaatcactcagcagctacttcaataaccatattttcgatttcagaccgtgataatacctacaaccgagtgtcagaggatctgagaagcagaattgaagtcctgaagcgcaaagtcatagaaaaagtacagcatatccagcttctgcagaaaaatgttagagctcagttggttgatatgaaacgactggaggtaagtatgtggctgtggtcccagatgtccttgtttctgagtagagggaaaaggaaggcgatagttatgcactgagtgtctactatatgcagagaaaagtgttatatccatcatctacctaaaagtaggtattattttcctcactccacagttgaagaaaaaaaattcagagatattaagtaaattttccaacggtacatagatagtaaatttcaaaagcaaatgttcagtccctgtctaattccaaagcccattacatcaccacacctctgagccctcagcctgagtttcaccaaggatcatttaattagcgtttcctttgagagggaatagcaccttactcttgatccattctgaggctaagatgaattaaacagcatccattgcttatcctggctagccctgcaatacccaacatctcttccactgagggtgctcgataggcagaaaacagagaatattaagtggtaggtctccgagtcaaaaaaaatgaaaccagtttccagaaggaaaattaactaccaggaactcaatagacgtagtttatgtatttgtatctacattttctctttatttttctcccctctctctaggtggacattgatattaagatccgatcttgtcgagggtcatgcagtagggctttagctcgtgaagtagatctgaaggactatgaagatcagcagaagcaacttgaacaggtcattgccaaagacttacttccctctagagataggcaacacttaccactgataaaaatgaaaccagttccagacttggttcccggaaattttaagagccagcttcagaaggtacccccagagtggaaggcattaacagacatgccgcagatgagaatggagttagagagacctggtggaaatgagattactcgaggaggctccacctcttatggaaccggatcagagacggaaagccccaggaaccctagcagtgctggaagctggaactctgggagctctggacctggaagtactggaaaccgaaaccctgggagctctgggactggagggactgcaacctggaaacctgggagctctggacctggaagtactggaagctggaactctgggagctctggaactggaagtactggaaaccaaaaccctgggagccctagacctggtagtaccggaacctggaatcctggcagctctgaacgcggaagtgctgggcactggacctctgagagctctgtatctggtagtactggacaatggcactctgaatctggaagttttaggccagatagcccaggctctgggaacgcgaggcctaacaacccagactggggcacatttgaagaggtgtcaggaaatgtaagtccagggacaaggagagagtaccacacagaaaaactggtcacttctaaaggagataaagagctcaggactggtaaagagaaggtcacctctggtagcacaaccaccacgcgtcgttcatgctctaaaaccgttactaagactgttattggtcctgatggtcacaaagaagttaccaaagaagtggtgacctccgaagatggttctgactgtcccgaggcaatggatttaggcacattgtctggcataggtactctggatgggttccgccataggcaccctgatgaagctgccttcttcgacactgcctcaactggaaaaacattcccaggtttcttctcacctatgttaggagagtttgtcagtgagactgagtctaggggctcagaatctggcatcttcacaaatacaaaggaatccagttctcatcaccctgggatagctgaattcccttcccgtggtaaatcttcaagttacagcaaacaatttactagtagcacgagttacaacagaggagactccacatttgaaagcaagagctataaaatggcagatgaggccggaagtgaagccgatcatgaaggaacacatagcaccaagagaggccatgctaaatctcgccctgtcagaggtatccacacttctcctttggggaagccttccctgtccccctagactaagttaaatatttctgcacagtgttcccatggccccttgcatttccttcttaactctctgttacacgtcattgaaactacacttttttggtctgtttttgtgctagactgtaagttccttgggggcagggcctttgtctgtctcatctctgtattcccaaatgcctaacagtacagagccatgactcaataaatacatgttaaatggatgaatgaattcctctgaaactctatttgagcttatttagtcaaattctttcactattcaaagtgtgtgctattagaattgtcacccaactgattaatcacatttttagtatgtgtctcagttgacatttaggtcaggctaaatacaagttgtgttagtattaagtgatgcttagctacctgtactggttacttgctattagtttgtgcaagtaaaattccaaatacatttgaggaaaatcccctttgcaatttgtaggtataaataaccgcttatttgcataagttctatcccactgtaagtgcatcctttccctatggagggaaggaaaggaggaagaaagaaaggaagggaaagaaacagtatttgccttatttaatctgagccgtgcctatctttgtaaagttaaatgagaataacttcttccaaccagcttaattttttttttagactgtgatgatgtcctccaaacacatccttcaggtacccaaagtggcattttcaatatcaagctaccgggatccagtaagattttttctgtttattgcgatcaagagaccagtttgggaggatggcttttgatccagcaaagaatggatggatcactgaattttaaccggacctggcaagactacaagagaggtttcggcagcctgaatgacgagggggaaggagaattctggctaggcaatgactacctccacttactaacccaaaggggctctgttcttagggttgaattagaggactgggctgggaatgaagcttatgcagaatatcacttccgggtaggctctgaggctgaaggctatgccctccaagtctcctcctatgaaggcactgcgggtgatgctctgattgagggttccgtagaggaaggggcagagtacacctctcacaacaacatgcagttcagcacctttgacagggatgcagaccagtgggaagagaactgtgcagaagtctatgggggaggctggtggtataataactgccaagcagccaatctcaatggaatctactaccctgggggctcctatgacccaaggaataacagtccttatgagattgagaatggagtggtctgggtttcctttagaggggcagattattccctcagggctgttcgcatgaaaattaggccccttgtgacccaataggctgaagaagtgggaatgggagcactctgtcttctttgctagagaagtggagagaaaatacaaaaggtaaagcagttgagattctctacaacctaaaaaattcctaggtgctattttcttatcctttgtactgtagctaaatgtacctgagacatattagtctttgaaaaataaagttatgtaaggttttttttatctttaaatagctctgtgggttttaacatttttataaagatataccaagggccattcagtacatcaggaaagtggcagacagaagcttctctctgcaaccttgaagactattggtttgagaacttctcttcccataccacccaaaatcataatgccattggaaagcaaaaagttgttttatccatttgatttgaattgttttaagccaatattttaaggtaaaactcactgaatctaaccatagctgacctttgtagtagaatttacaacttataattacaatgcacaatttataattacaatatgtatttatgtcttttgctatggagcaaatccaggaaggcaagagaaacattctttcctaaatataaatgaaaatctatcctttaaactcttccactagacgttgtaatgcacacttatttttttcccaaggagtaaccaatttctttctaaaacacatttaaaattttaaaactatttatgaatattaaaaaaagacataattcacacattaataaacaatctcccaagtattgatttaacttcatttttctaataatcataaactatattctgtgacatgctaattattattaaatgtaagtcgttagttcgaaagcctctcactaagtatgatctatgctatattcaaaattcaacccatttactttggtcaatatttgatctaagttgcatctttaatcctggtggtcttgccttctgatttttaatttgtatccttttctattaagatatatttgtcattttctcttgaatatgtattaaaatatcccaagcaa

SEQ ID NO: 3 - DNA, 78 bp, Homo sapiens
  source 1..78: mol_type = other DNA
ctgaggagcagggcttagctgcttgtgagcagggtccacaccaagtcgtgttcacagtggctaagttccgccccccag

SEQ ID NO: 4 - DNA, 23445 bp, Homo sapiens
  source 1..23445: mol_type = other DNA
gtagtctctttggaaacttctgcaggggaaaagagctaggaaagagctgcaaagcagtgtgggctttttcccttttttgctccttttcattacccctcctccgttttcacccttctccggacttcgcgtagaacctgcgaatttcgaagaggaggtggcaaagtgggagaaaagaggtgttagggtttggggtttttttgtttttgtttttgttttttaatttcttgatttcaacattttctcccaccctctcggctgcagccaacgcctcttacctgttctgcggcgccgcgcaccgctggcagctgagggttagaaagcggggtgtattttagattttaagcaaaaattttaaagataaatccatttttctctcccacccccaacgccatctccactgcatccgatctcattatttcggtggttgcttgggggtgaacaattttgtggctttttttcccctataattctgacccgctcaggcttgagggtttctccggcctccgctcactgcgtgcacctggcgctgccctgcttcccccaacctgttgcaaggctttaattcttgcaactgggacctgctcgcaggcaccccagccctccacctctctctacatttttgcaagtgtctgggggagggcacctgctctacctgccagaaattttaaaacaaaaacaaaaacaaaaaaatctccgggggccctcttggcccctttatccctgcactctcgctctcctgccccaccccgaggtaaagggggcgactaagagaagatggtgttgctcaccgcggtcctcctgctgctggccgcctatgcggggccggcccagagcctgggctccttcgtgcactgcgagccctgcgacgagaaagccctctccatgtgcccccccagccccctgggctgcgagctggtcaaggagccgggctgcggctgctgcatgacctgcgccctggccgaggggcagtcgtgcggcgtctacaccgagcgctgcgcccaggggctgcgctgcctcccccggcaggacgaggagaagccgctgcacgccctgctgcacggccgcggggtttgcctcaacgaaaagagctaccgcgagcaagtcaagatcggtgagcgcgctcagtgtgccagtcagttacgcggcgcacgggcgggggacacgagaccggctgggcccgcgcgctttgcgcagcaagtggcttcgagctggggtgcagctcgggagtagtcggggagggtccttgcaccccggaattggagccctggaggatcctgctacccgggggaactgtctagccgagtctatcccagctttcgctctttctccttcctcctacccacacgttgcccgccccctccccctactctgtccgaatactgattctgagctcttattcggtcacaaggtccaaatcccctggtaccctatctacagtctgaaagagtgtatgttacattatcaactccctcctccacccccctcgcgccccgcataggtttttttctgaacttggaaaaaaaatctcttttgttaaaatattattttaattgcggcctggagagagaggcattacctatcttctgagctaattccacctttgtccctcttggcccctccacccccgtgcctccagacgtttctatccctccacccctacacacacaccacaaacaccccacatccttggtagctaatgcctttcgggtgggagccctgaagcccctcccatgtgcataaccattgctttttattgaagatgattgcctgtggtagatggtaaaacatatttaactgcaaaatgacttttattttatcccaggaagggaaaaaaatactttaggagtgcgggggtgcggggtgggggtggggaagagtagaaaggaagggtttggtattctgtgcctggtgttcgtttctgaatctaattccttttccccctctccaattcagattttacctaggatgaaaggtggacatagggctgggaggcaaaaggggatgtgagattcagagctttcaacttcctcgcctatgcagattcctggcaccaccaccacctccacccccgccccgcaattcctccctccgcaatccccccaccccgccctccccaatctcttaaaccagatcacaagtgggtgtggattaagtgcatgaggggccctggaaacgcagaatgcaaaattcagggggcggagacagaaaagccacgcactgggagcctcgcctccgcttgccccgcccccgggttgcgccgcccccaaattctcggcgccaggagtctagggttgaaatgattgacacagctacttgttcaatcagaacagttctacccccttagactgagtttctttttggaaagagttacctgatctttagttaaaaaaaaaaaaagttaaataaactacataaaagtctgggttctaagacgtcaaactggctattgattctctccaaaaggggttaaaacttggctaaacaatgtttatttggcgtagtttagttacggagacagtttagttacgggggcaatccccttctccctccctgtccctttccgttactcacgagcaccctaacatgagttttctgaagtgcaaatttcagtcactatagtgcaggagaggagtgcgtccgcgcttgccaggaggccggagagcttcctgtgttcagcctcagtccccgcaaaccctgcagggtttgagtggcgcaggggccagcccctctagctttgcaagaggtagtcgatctccaaacctgcaaaaagtcgatctttttgcaggttgcagcctgcaaaaagaggaaaaggggaggatgtgcaggctctgggaaccccagagaccggcttgtgagattatttttattaagatccacttttcaaaggcggtcctgcccgccttcatcttgggggatgtggatttggaaaagcctagcggagaaggaaaacattaattgatttcccggcttgggagccaccgccctgggtaacaatccagtcacaccgaaagaacgtaaggtgtcactcagccgcatcctggctccacttattatttaccaagcgtgtagtgtgatgtggctagtgtgaagggtgtacacgcagagcgcacgcgcgcgcaattgctaggcgagcacggagggcgcatcacacacacacacacacacacacacacacacacacacacacgacacttcagtcccaagcaagatcccctgtagaattccctgccgccccttgctcaacccccaccttctgagtgcctttgggccaacccgaagccgcctcttctacccgccccctccccagcactcctctccgactccaccccgccgaaggcaggtgcccggccggctgctgttgcgggttggcggcgctccaccgctgctggtgccgacatcttcttcccgaacagatgggatgggagtgggcgctcctggaaagggcgttttagccggacaaccactgggcgggtccccaaaaagttggagatggtgtagagaccgttcttaaggagagagaaatggacagagagagggagagtgcccttttggtcctttagccaaaattcctgcttcccaacacacctcctacctccctcctctcccccacccccgccaaaatctgagcttgcagatatggatttgccccctccctcccgcagttgcagcatacacacacacacacacacacacacacacacacacacacacacgacatattatatctatataattatatattgtatatatggtatatactatattatatatatttatatgtaaccaaacatgtagaacccaaaaaaggtgcatttctggaatcagaaatggggagcagaagagagtgaggtggcaggcagccaaagcctctgggagggaaaggagagggcggaggagagggtgttttgctaggctgttgctgagcaactggagagggagtgggcccgagagcagggtgctgagagcgagcctggctctgcatttcattctggccagttcaggagcagagatagatacggaaaaaagaatgtgtgtgaggctggagggagatgaaagacgggagttatttgatgggcaaagctcagtaaatagcggtgagtggagggagtcaaggaagtactgggtttgctttcgggcatttttggtggggaatgaggtttgatgggctggtccccagcatagataccggggttcgggtaggtctcctctgtgctggtgagacattcagtttaagatgtagggagccgtgggttctggctttcggttctgtcattaagaaatgagacaccgtgggacaaaaaataggcttctggaaaagaaagcaaaagcattacctaaataaaagtgaattcagcctttgcttctttgaggggtttggcctccatcaccctggcttcaactccaagcctggtctaaaatgccatgttgaagtcgagttccagagttaggtttattggccaaatttatgtctgggttgagcaagatcatggaaaactgaaggagccaaattcctttcccacccgcaccccctccctctgaaacaagtctttgagaggatggcgtgccctgagccaaccaaaacgggagttgggaaaacgagatggggctttaactggacttttctcgccacctccgcccaccgcccccgcccccgcccaccccgccccccctcccccacctttctgctgtgtcagctcagactggaagaacaagcagagttagccctagtgagagctcatattctttccatttctctttttcccctttctcacccctccctcctactcttccctccgaccttctccatccaccccccgaccccccaccccaactctaaggcatcccctgagggcttgagttttaagtcagagcagctgtgagttagtcccggggcttgggctggatttgagcaggcaggtgggcctgcagctgcagagggtggaccagcctgaccctaggagccagaggtcatcgtgagggttacagcaaagggcatgggagcaggaattccctgcagaagccctggcccccttaatggagcgaagaagccagcgggaagggaaggtaatacttgtctaaagtttctactttgtacctgagcaatgcctatgaaacttttaagatatttagtgtgtggaaaataaaactctggagaagagatcaccacactccagacccactacatccagaaactggaagaagatcataaagagcaggtaccaaccaggggccagagcagaagggaagagggtgggagaatggctgcgttgagtcaagcaggcgatttggaggggtttgtttagttttacatttgctttttctctacagttggtccaaaagctgcaattcccagagactatccttaaattgcaatcaggacatgttattcaaaacagtaagactgattacacattgattacatacttgcaaaaataaataataaaataaacaaggatggcagtgtaggcttctactcccctcccccaataccagtgaaatcccccccttttatttccagtttcatttctttccataaattctgttatgatgtcatttctctctctctctctctttttaaaaaatataaatccagaggagtgactgaaaatctctgtgaggaggagaggttatattcccaccttggccactatgctgttggtttagagcacctaaccaggttagttagttagtgcctggccactcagcttagctcagtcctagtgtctctccaggaattgtctgggtattggccaaataatgttaaagctggaaggaacccatagccatcatcacagtcaaggtcctagttttagaatgaggatactgaggccctgagtgggaagtcacttgcccaagatgtggcagcagggttagagacagacaaggggctgggactcagctctttcccgcaggggctccagcactgcattcagccattcctggctttctcgctagtcactggggctcatgcctggacctgggctaacctgcagtaaggcctttggcaaacactgccagatgctatcactccatgacataagaacccataatctgaaggcactctgttttaggggcagtaggaaaaggagtgaagcggccccaaagtggagagggccacactctcttattttcacactcacttctgtccctttttctacacagtcttgcatacaagcctggcttaggctagtggtttggtcagagaaagaggaccaagagggtgtgaaggaggggtgttcaccccagctttcaggtccatgcgccaaacctcattttctacatgacaggaagctctcctgatgtggagaggcaggcaggcctggctgcctctgagctgtgcagcggcctgtagtcttgaagaacatggtgcagaagtggcccgcttccaacagcacagtcctcacgtggtgccaacagaaagcagagatcgagagagggtgtggttggatggggtgagtgcagtaactaggaagttctgcatccgaaggagagaaggaaaaccatataccaccaaagctgataaggaagagagcatgagggccccctggctttctttcataggcagatgtgtctcagatctttcagcaggagaggagagatgtgcttccagagggcagctggggacttctggttgtgctgcaggaagtgctgagacccattctaatacatcctggaggccgtggcagctcctccttctgggatgcttaggaaggaggcagataagataggcccctttttccggtaagtcagacctgccaggtgaactataggaacattttaaacgaactcagttatctcatgtttgatccctcaacctaaaccatcaggcccctttccctggcctaaaataaggtcccactgaatctgcactcagagccaggcctcagatgacctctgctgattctctgagttgtttaatgtgggttccagttatcccgaactgggactgcgacacccctctgtcacctcagccaggatgactcttcttccagatcatttagaacagcacttccaattgaaacataatacaagccatatttgtcatttttaattttctggtagccacatcttttttaaaaaggtaaaaaaaacagggaaattaattgtaataatacattttaactgaatatatccaaaatatcctttcaccacacgctcaaaataaaacaattataatgagatattttacattctttccttcatatttagcctttgaaatccggtgttttttacacttacagctcatctcaattcagacactaaattttcattggaaatacttgatctgtatttagatttcataaaatttacagttgaaaaagcagagtcacatacctgaggcattccaaacatactttaaaatctttccaataactgagttgagtatctgtttttaaatttaaactaattaaaattaaataaatattaaataaattttaaaatgtggttcctcagttccccgggccacatttcagatgttccgtatgtatctgcacatggttaatggctaccagcaaacccctctctcacctgagaaggcaactgctgtccccactctttccttttgctcccaaagactcaaaaaaggggagtctcagctttcgttgacagacagggctcccttgtttggtccctagcagagcctgggcaccttcttcggggcctcaggagagaagcgtaaaccctacttcctccctgccgcccccttctggtcatgcagaactttggggggatgtggctgtggctggcaatgttctgaactggctgtgatgggtcatgatgggaaagtggccaggagaaaagctgcccagtgcttcctccagaggctgctccccacctatccccccaccattaccttctcatttggggaatgtatgaggaacagacagacacttctactaagcatgctcccccttccccaactccaaaagaagcttggctggagattctcagccagggacttgtgcatcagtgtgtatttcctatgtgtacagttatcgccagctgcttcccagggaccaagaaatgtgaaccagagtcacaaccccaaatcctagtttggcatcagaaaacaacaaggagcctctctttacctctggtccctggacagtggggcagatgtaagggggacctcagccccttactctgtgaggtgtcaccttcccacctgtggcatctacactgtggagggcggtgggcccccttttctctatatatcttcagggaaggaggctaagtgcccttaacgcagcatgaaggaatggggttaggcagaggaaggactcccagggggagctctctaagtggagacgggtccggagagcacctgtgccaagtcctcacctggtgttggccaacagacccccagagacaaaggtcgagccaacactttctggcagaccttcctgcagtccaaggagcctcagatcttgtggtctacaagtaggcgtctgtcaaccaggtgtcacagcaaccaaatttttagttgatgattcgaactagggaggtggtaggaaacagcactacaaaggcagagacctgttctgagagtgaattagcatgcatcaccctgattaatcctcagaatataatggagaaggggccattgccatcctccccataacacaggtgagaaaactgaattggaaagaggaagaagaaagtaaggtctttgggaggctgaggtgggtggatcacgagctcaagagatcaagaccatcctgggcgtggtgctgcatgcctttagtcccagctactcaagaggctgaggcaggagaatcatttgaacctgggaggagagggttgcagtgagccaagatcatgccactgcactccagcctggcgacagagtgagactccgtctcaaaaaaaaaaaaaaaaaaagaaaggtcaaagtaaatctgtaccaaggtttgtttatttatttatttttagaaacaaggtctcactctgtcacccaggctggagtgcagtggcacaatcatggctcactgcagcctccaactcctgggttcaagccatcctcccttctcagactccccattgctaggactataggtgcacactgccacgcccggctaatatttcattttatgtagagatggggtcttgctgtgttgccaaagctgcatcaaggtttactgagctattgtcaacagcttcatcttcctcccagaaaggacagctgaaggtttagggtggcacagtttgctgtacctattcagtagtggagctgggatttgaacccaggtggtctggttcctgattctgaatggttatccactatactacatggtgtctgtatttctctggtaaggatagagatatattcccagcttggccagctttgctgttggtttagagtacctaaccatgctatttctcccggcctaaaatggggtaggggggctcagctgggtacacctatagccctcatcatccagtcagtagttctctaagtctgctcaactcccctccggggtcttcctcctggctttcctccattcttacagctgctttttaggatgacagctttgggttttttttttttcttaaaaggttagtgctcatttcctcctcagcccataattcaggttaaaaagaacccggaacatgcatgcctatttctgacgatcaagtaaaaacaaaaacaaacaaacaaaaaacaaaaacaaaaaaaaatgtcttctgagagagactggcgccaggcagctgctggtcagagatgggatgggtaggaaaagaaatgatgttgccacttccctggaagtgtccacagcaccttccccctgccacaaccactgtggcctttctccttctgcaaatgcacacacacaagcgcagaaaagccatttgacatccacagctgggaaacagacttcaagagactgagacatgtcttacattttttcaaacagtgaacagccaatccctcatgcttccaccagccttgtgttgtagggaggggctggtggctgcaagttggctagggacctagggttggcaagggaggagggggactgcagaacattctagactgggcctcagtattttcatccatacccaggcacaagtcagtgccgtcaggccagcactgaccaggactttctgcaatgatggaagcgttgcaggtctgcaatgtccatatgtggccacgaagtccttgaaatatggctagagtgactgaggagctgaatttttcattttatttaatatttatttaaatagccacattggctagtggctaccatattaaatatatacttttttttttttttttgtcacactattgcccaggggggaatgtagtggcacgatcttggctcactgcaacctccgcctcccaggttcaagtgattctcctgcctcagcttcccgagcagctgggattacaggcacacaccaccatgcctggctgattttttatttttagtagagacagggttttaccatgttggccaggctggtctcgaactcctgaccttgtgatccaacctccttggcctcccaaagtgctgggattacaggcgtgagccaccatgcctggcctaagtagtacattaatatatagtagccttaggccaaagagaagcccagtgaatccaggagcacccctgctgtttctcacacccatgacgctcatctgtctgcttccctgtgccctgcggcagggttatcttgctccagggcaggagcatggatgagataacctcccaaggcatgcactgggctctaagccccagcttatattacagaaatacttccagacctacttctctttgcctcttgggcagatttacacatctctccatttaaaggttatttattgaatactatatgctggtgagacaaagagaaatgacaaagctctgcccgtaagaagttggctgtttaaattccacaggggggactagaatgaaacccagaacaaattcagctccctttttcattctttgtagagagattctaggcgtcctcatcttatcttctgtctagaaaaggagatgggagaatctccccaggtctgggtggcctggcaaagcccgacactcttcctggactgtgaatttcaaggatgcctctgtttcttcgatttttgtaagctaaggcacaatatctgggtcacctagttttctcttacaattgattattaggtcaagtgagatagagtgataaactaacaccagcccaggaacaggctgttaatagcaccggggtgtggctaagaggtccgggggcggggggtttagattttaggcaggcaggtctcctggatccatccattgctgtgaccagcaagcaaggtggagtcagaacccttcagactctactggaagagaacagccgtggcaaaagggcaggtttggagaaagtggttgagcttgggcagggtacatgcgttgtgcaattgtgcagcatggagtatttctcaccctaagatgcctctgggtctgtagcagctgggcttgcatcatgacactctctgtgtttgccaggacatagaggatggtgcaatcctcaaacacgtgttcatgttaccatggggagaggctgatgtactgtgtgtgcctctgtggatgctgctgcactggggtgtatggggaactccttatgaatgaaagaggactgagttggccacccaaatgtggcaggggccagaggcattggagagccagtgggaaggactggaggtattatatagaagccagagatttagatcccaccccaaaggtaaatactgtatccagataatattatcatcatcccctcccttagtcattgaatagggttatgaaggtaaggtctggcctccatagatcccagcaggagaaatggatgctgagcattccacatttcccatcctctgcaaaaacctctcagaacagcatctcatgggcggggaagtctggaatatgtctctcttccttcctggatcattttccagttggaggttacagaaacagcagaatgccatgcacaaacaagccctgttcccctctccctcacctgccttcactctcccacacatgggttctctccgggcctcgcttgtttgtctccctgactctttaaatatatcctgcagacacacaaacagaaggaagggatttatttgaatgattattgcagaagtaggagagggaggcacccaaattccagatttattttttctttgagacagggtctcactctgtcccccaggctagagtgcagtggagctatcaaagtggagcaatcatggctcacctcagcctcagcctcaacctccaatctccaacctcctacctccaacctcccaccttccgggctcaagcaatcctccggtctcagcctcctgagtttctcagactagaggcgcacgcctctatgcccagctaatttttgtgttttttttgtagagacggggtttcactatgttgtccaggctggtctcgaactcctgggctcaggcaatccactcaccttggcctcccaaagtgctgggattagagatatgagccaccgctctcaattccaaattccagattttaaaaacacttccaggccgggcttggtggctcacgcctgtaatcccagctctttgggaggccaaggcgggcggatcacgaggtcaggagatcgagaccatcctggctaacacggtgaaaccccatctctactaaaaatacaaaaaattagccgggcatggtggcgggcgcctgtagtcccagctactcgggaggatgaggcaggagaatggcgtaaacccaggaggcggagcttacagtgagccgagatcgcgccactgcactccagcctgggcgacagaaggagactctgtctcaaaaaaaaaaaacaaaaaacgcttccagtccctagaagtgtgcccatgctgtgtgggtgtcagtctcccacgccctctgctggccacatggagatattgacctgtttgtcaaacaggttccagagcagactgttgagttcttttgctgttcacgtgcagaacaatcttcaccaggaagtcctcccgggtatcctgcctagatcccttctgcaacctcagttcattttctcttgatgaaatagctccagagtagccagtctacttgttccttcttgttttatctaaaacgcaaagccttccacaattgaaagcctatttatgactcagccacagagcagctgagtcgggctggctgcttctggcactcagctccagtcttactttccagccctttaatctccatggctctgccctggctcccctccaagtttccgctgtctctctggagcctacaggtgaccacaagaccctgattagtatcttcgacactggactctgctgctgcctaaggaataggtcccatggggttaagtggcaccagaaaccaggaggcacatcaaaatgttaagcctgctcttcagaagcagccaaaaagcttgcaaagctggggaaggtgtgccctcaggagacttgccttggggaggctgggaaaaggagagagtttgcaaaagcattttgagttccttaaatgaagagagatacaagaatctacattttgtatgccagtatcatggttgcttggccccggggcagtacttgaacactttcaaagaaaagagtaagagaggtcaaaataaatttaccccaaggtttatcaaaccgttgtcaacagccccatccccctcccagaaagggtgactcaaggttaaggacagcccacagcacttcttagaaaaagtcccaaaaggtgaaaggtcttgagaagagctgttgagggaaggctgtgggccaccatgcttctgtgtcccccaaggccaaagagagaataagctaaaatgacagctggaaaagggcaccctctgaccaaatggacagagcctcccccaacaggtagccagaggaggatggaatggcacccccatttcagatgtccttaagaactagagagatagatgcttatttctgcttggacacagggggatggactaaatggcctacggaaaggattccaggaactgctacaccagccacaggagagaagccagcttcccaggctgtctccccttgaagaggtgacaatgtgttggctctccaggccaggctggggcagcccactgaaggagacgcatagacgcatgcgctggtcagcagccagcccactcccccacctgccctcactttatccagttacaatcttgattgaggaaggggtccaggcttctccaatctgaaccccctccaggctttcagtagccaccatatcctgtctgcccctccccctacagtagtcaactactttttgaggattaaaatgcgtggtgatgctgaggttgagtggcacggctccagtccctccataagacgtgcccaaaagcccttctgtgcaatggttagcactccctctccctactccctcttctccaagatctgagccttggcgtgaggcctgtgttactagataacggagccccagcctttcaatttgtacaaagtccccaaaccagccatgcttctcccttcctcctgccaatctcacttgcgctacaaccaagaaaagtcaatttaccccagaacatgacccttttaactaatccctagaatcctgcattccacctaccagagatgtcaccctattgatgagtcgtcacagcagggtctgatagagcagaatcgaggtactgggacatcaagacatgactgggaagagggggtgagagtccagaaggggtaccaggattctcaggttgaattttatttagggagagcccacccaccaccttgctatttgctttccccaagtcatcatcttcctctccagtaattacgtcccttcctttcctgtgaataaatacccaaagcaactcaccaccaggaacgctgcgaacctttggaggcttctttagggcagggaccttctctgccaaggccttaaagaccagatacctatttcattagacttgacaaatcctgagccaagagagaaacagatgcttgggtgcttcctgccacctgccatcctgcccaggttaggccaggtgtccaaatgcctttcctaactcacacctggaacttgcccagggctgcaagctcagaagtcaggttctatacctgcccagaggcataaaacagcgtcttctcaaaaaagcttctctttccttgcaccccacccccacttcctggaattctacccacttcttctgttccccatcccagatgtctggcggtcactgttcctggacatcccagtgatcatggagtagatggagaacagaattttctttcacctcatttcagttatttaaggtcactcaaagctctattttctctttccagtatttgaaaaaagagggaggcaatgaagacagggccccccacctccactcacccctgcatctggtcccactgtgaggcatcctggccacacgctgcccgcctggaaacaacaatctaaagttcccccattctggttcctctgaggctgggggaggtcaaggatctgagaggagaaggggacccagggatggatgcctatgagatcagaatttaggggaaaactgcgcaccaagaaaaggccggacgggtggaattaaggatcaacaaatacatcaacaaagtctgacttctctaaaggtcaaaagccagctaagtatagactgtcagcaagccactcctatatataactgtcccggtctcagccagctgtcggcctctctcagtccagagctgagtaacgtcccagcctcccaggcccccgagcaccgcgccagttctgagccagagcaggagcaaggcctccgacttccacttggccccacgccggtcccctccgggcctacatttctggctctcccctcccctcctcctgccgcttatgaaggtcctcaccaccctgctgctccagaccccaggaccccctcctcctaggttccccaggtccaaagagacctcaacatccagcagctctgaaagtgcaaagatctcactaacaggacagcctttgcccttctcgtccacgccctgactgtgtcatctgcctccatgggcccagattcccgggttcctacttctcagccccacctccagccatgtcccatctacttggccatcccccagcaagcaaaccgctcgctgccaccttcatccttgcagaggccattttccttgcccttcctccttactgcccccagaaggcctgctccgtcctcacccatcagtctgtcagtctctcgattctcctcctctgtgaagcctccctgcctgcactctctgcttgactccaagcatgccagaaacttcctgccacttaaatgagcattccctctgcttcctggttcttatccccctgctttcagggtgtgctccaggagggcagagacacatctgcttcagcctttattactcccctcaccccaaactgcccagccctgggctctggccgtgtgcaccttggcccacgggggctgaccctccggctccttctcctgcagagagagactcccgtgagcacgaggagcccaccacctctgagatggccgaggagacctactcccccaagatcttccggcccaaacacacccgcatctccgagctgaaggctgaagcagtgaagaaggaccgcagaaagaagctgacccagtccaagtttgtcgggggagccgagaacactgcccacccccggatcatctctgcacctgagatgagacaggagtctgagcaggtgcatctcggggattccctcattccctcccagcttttgaccttttcctgcatctaaatggacattcatggcggcaggaggtgctagactagacccagcagaggacctacagcccaccatgtggctcagcttaggacgtgggagtagagtttccagagcatacacttgtcagggccaagggcttgtgcaagtaagtgggaatagaggcggtgctcatttgaggagagtgtgtgccagcccagcggccacgtaccaggtacctgggccctgcagctgtgtccagtccaaggcagagactgaatattctcctagagcatctagaaatgggcacctctggacattgttactcagcagaagagaaaagctgcaggggagggggtggactggaacacaaaagagaaagtatgactccgtacctggccaaaggcaggctttgtatgatcccagcgcacgtgacaggtgacagggaggaaagatctttggtagcagatgattagaaccaaaggtggtgactttcctccagagacccttcagcccccaccccctgggccattcgtcagcgcagctgggtggttttcccttggtctcgccacgcctctcaccctcctgtccacacagggcccctgccgcagacacatggaggcttccctgcaggagctcaaagccagcccacgcatggtgccccgtgctgtgtacctgcccaattgtgaccgcaaaggattctacaagagaaagcaggtacgtcccctgccctgagctccaggctcagactgctccaaaaatggcacctgccaggaaactccaccttgggcaagtgcctaaggtttccaccgttaaccacttagtgtttcctgggcctcagatacccattcatataccacgatcatgactttccacattccctactatgctgtaatccatttcctcattctctcctatgcggtaatccactatgctttccacaggtcgccttagctacatgaattccttgcaaaaggtaactctgtaacactatcgcacagcacgtatcattggtgcaccgcacactcaggaatttaaaccatattttctctgtgaaccacctgaaatcagttcatgtcccttcacagccaggctctcctttgggcaatggttcttagatttccaagggcatcctatccctggagggcatggctgatggctgggccccacccctgcagtttctgattggtagacctggggtggactccggggtggacacgtgaccctgatgctgctttaagggcaccaataatctaaatgtaagagccaggccacactggggcaaatcttggctctgccacttactagctgtgtcctgttactcaccatttaatgtctctgtgcctccagacccttgtgtaaaatggtgaatgaggagtgagtgattggtctttgtaaagcacttagaacagtacctactgcctaccaaacgttgagtggtgtctactacatgataacaccacaaatcatgcctccttctgttattattattaccatcatcattattattggatcataactctcttgagaatccctgcagagtttcacgttgggggaactcaaatgggtaatatttaaaacgggactataagccaggcacagtggctcacgcctgtaatcccagctactccagaggctgaggcaggaagatcacttgggctcaggagttttagaccaacctgggcaacataacgggaccccatgtctgaaaaaaaaaaaaggaaagaaagggattgaaggagcttgccaagggtaggctgcctaaattcacattttccctgggtctttccgtgaaatggggacaccagaaacccaagggtcgggtctagtgccctcaactctctggggatgagagtcttgccttggggtagacaagaggcagggcagggaggagcagagccctggggtgcggccgtcctcaccgcctgttgctctactcaccccagtgcaaaccttcccgtggccgcaaacgtggcatctgctggtgcgtggacaagtacgggatgaagctgccaggcatggagtacgttgacggggactttcagtgccacaccttcgacagcagcaacgttgagtgatgcgtccccccccaacctttccctcaccccctcccacccccagccccgactccagccagcgcctccctccaccccaggacgccactcatttcatctcatttaagggaaaaatatatatctatctatttgaggaaactgaggacctcggaatctctagcaagggctcaacttcgaaaatggcaacaacagagatgcaaaaagctaaaaagacaccccccccctttaaatggttttctttttgaggcaagttggatgaacagagaagggaagagaggaagaacgagaggaagagaagggaaggaagtgtttgtgtagaagagagagaaagacgaatagagttaggaaaaggaagacaagcaggtgggcaggaaggacatgcaccgagaccaggcaggggcccaactttcacgtccagccctggcctggggtcgggagaggtgggcgctagaagatgcagcccaggatgtggcaatcaatgacactattggggtttcccaggatggattggtcagggggagaaaggaaaaggcaaaacactccaggacctctcccggatctgtctcctcctctagccagcagtatggacagctggacccctgaacttcctctcctcttacctgggcagagtgttgtctctccccaaatttataaaaactaaaatgcattccattcctctgaaagcaaaacaaattcataattgagtgatattaaatagagaggttttcggaagcagatctgtgaatatgaaatacatgtgcatatttcattccccaggcagacattttttagaaatcaatacatgccccaatattggaaagacttgttcttccacggtgactacagtacatgctgaagcgtgccgtttcagccctcatttaattcaatttgtaagtagcgcagcagcctctgtgggggaggataggctgaaaaaaaaaagtgggctcgtatttatctacaggactccatatagtcatatataggcatataaatctattctttttctttgtttttttctttcttcctttctttcaaaggtttgcattaacttttcaaagtagttcctataggggcattgaggagcttcctcattctgggaaaactgagaaaacccatattctcctaatacaacccgtaatagcatttttgcctgcctcgaggcagagtttcccgtgagcaataaactcagcttttttgtggggcacagtactggatttgacagtgattccccacgtgtgttcatctgcacccaccgagccaggcagaggccagccctccgtggtgcacacagcacgcgcctcagtccatcccattttagtctttaaaccctcaggaagtcacagtctccggacaccacaccacatgagcccaacaggtccacgatggatccaccagtcccaccccagccttttcctttcatctgaacagaatgtgcatttttggaagcctccctcactctccatgctggcagagcaggagggagactgaagtaagagatggcagagggagatggtggcaaaaaggtttagatgcaggagaacagtaagatggatggttccggccagagtcgatgtggggaggaacagagggctgaagggagagggggctgactgttccattctagctttggcacaaagcagcagaaagggggaaaagccaatagaaatttccttagcttccccaccatatgtattttctaggatttgagaggaaagagaggaaaatgggggaatgggttgcaaaatagaaatgagcttaatccaggccgcagagccagggaaggtgagtaactttaggagggtgctagactttagaagccagataggaagaatcagtctaaactggccatgctttggaagggacaagactatgtgctccgctgcccaccttcagcctgcaatgagggactgaggcccacgagtctttccagctcttcctccattctggccagtccctgcatcctccctggggtggaggatggaaggaaagctgggacaagcagggaacgcatgattcagggatgctgtcactcggcagccagattccgaaactcccattctccaatgacttcctcaaccaatgggtggccttgtgactgttctttaaggctgaagatatccaggaaagggggcttggacactggccaaggagaccccttcgtgctgtggacacagctctcttcactctttgctcatggcatgacacagcggagaccgcctccaacaacgaatttggggctacgaagaggaatagcgaaaaagcaaatctgtttcaactgatgggaaccctatagctatagaacttgggggctatctcctatgcccctggacaggacagttggctggggacaggagaagtgctcaatcttcatgagacaaaggggcccgatagggccagcagccacaaggccttgacctgccgagtcagcatgccccatctctctgcacagctgtcccctaaacccaactcacgtttctgtatgtcttaggccagtatcccaaacctcttccacgtcactgttctttccacccattctccctttgcatcttgagcagttatccaactaggatctgccaagtggatactggggtgccactcccctgagaaaagactgagccaggaactacaagctccccccacattcctcccagcctggacctaattcttgagaggggctctctcttcacggactgtgtctggactttgagcaggcttctgccccttgcgttggctctttgctgccagccatcaggtgggggattagagcctggtgtaagtgcgccagactcttccggtttccaaagttcgtgcctgcgaacccaaacctgtgagtctcttctgcatgcaggagtttctcctgggcagctggtcactccccagagaagctgggccttcatggacacatggaactaagcctcccaaatgggagttctggctgagcccagggtggggagatcctgggaagggaggcactggaggaagacggcacctcttcccccatggcagggtgtgagggaggcaggtttggaatggtgcgagtatggcaatctaagcaggggtctggtctctttgactccaggctggcctttggccgactgtctgctcacccagagaccttggactccggactatccatggctccgaatctaagtgctgcccactcccatgctcacacccacagaaggtcttcccatcccctttagattcgtgcctcactccaccagtgaggaagatgcctctgtctttcccacgactgccaggagatagggaagcccagccaggactgaccctccttcctccagcctgccctgacccacctggcaaagcagggcacatggggaggaagagactggaacctttctttgacagccaggcctagacagacaggcctggggacactggccccatgaggggaggaaggcaggcgcacgaggtccagggaggcccttttctgatcatgccccttctctcccaccccatctccccaccaccacctctgtggcctccatggtacccccacagggctggcctcccctagagggtgggcctcaaccacctgctcccgccacgcaccggttagtgagacagggctgccacggcaaccgccaagcccccctcaaggtgggacagtaccccggacccatccactcactcctgagagggctccggcccagaatgggaacctcagagaagagctctaaggagaagaaaccccatagcgtcagagaggatatgtctggcttccaagagaaaggaggctccgttttgcaaagtggaggagggacgagggacaggggtttcaccagccagcaacctgggccttgtactgtctgtgtttttaaaaccactaaagtgcaagaattacattgcactgtttctccactttttattttctcttaggcttttgtttctatttcaaacatactttcttggttttctaatggagtatatagtttagtcatttcacagactctggcctcctctcctgaaatccttttggatggggaaagggaaggtggggagggtccgaggggaaggggaccccagcttccctgtgcccgctcaccccactccaccagtccccggtcgccagccggagtctcctctctaccgccactgtcacaccgtagcccacatggatagcacagttgtcagacaagattccttcagattccgagttgcctaccggttgttttcgttgttgttgttgttgtttttctttttctttttttttttgaagacagcaataaccacagtacatattactgtagttctctatagttttacatacattcataccataactctgttctctcctcttttttgttttcaactttaaaaacaaaaataaacgatgataatctttactggtgaaaaggatggaaaaataaatcaacaaatgcaaccagtttgtgagaaaaaaaaaaaaaagccgaaaaaaaaaaaaaaaacacctgaatgcggaagagctcggctcccgtttagcattttgtacttaaggaaataaaaaaccaacaaaggatctcacattttcttaaaaagtgaagattgctgtatactatttattcaacttataatttatgttactccttgatctttgtcttttgtcatgacaaagcatttatttaataaagttatgcattcagtta

SEQ ID NO: 5 - DNA, 66 bp, Homo sapiens
  source 1..66: mol_type = other DNA
aaaaggtggatattccttctatgtttatgttatttatggttaaacatagaggaaattccacgtttt

SEQ ID NO: 6 - DNA, 110 bp, Homo sapiens
  source 1..110: mol_type = other DNA
atcattcagaaatggtatacaggaaaatgacctatgaattgacagacaatatagctgagtttgtctgtcatttctttaggccaatattctgtatgactgtgctacttcaa

SEQ ID NO: 7 - DNA, 13889 bp, Homo sapiens
  source 1..13889: mol_type = other DNA
agagtcctgagctgaaccaagaaggaggagggggtcgggcctccgaggaaggcctagccgctgctgctgccaggaattccaggttggaggggcggcaacctcctgccagccttcaggccactctcctgtgcctgccagaagagacagagcttgaggagagcttgaggagagcaggaaaggtgggacattgctgctgctgctcactcagttccacaggtgggagggacagcagggcttagagtgggggtcattgtgcagatgggaaaacaaaggcccagagaggggaagaaatgcccaggagctaccgagggcaggcgacctcaaccacagcccagtgctggagctgtgagtggatgtagagcagcggaatatccattcagccagctcaggggaaggacaggggccctgaagccaggggatggagctgcagggaagggagctcagagagaaggggaggggagtctgagctcagtttcccgctgcctgaaaggagggtggtacctactcccttcacagggtaactgaatgagagactgcctggaggaaagctcttcaagtgtggcccaccccaccccagtgacaccagcccctgacacgggggagggagggcagcatcaggaggggctttctgggcacacccagtacccgtctctgagctttccttgaactgttgcattttaatcctcacagcagctcaacaaggtacataccgtcaccatccccattttacagatagggaaattgaggctcggagcggttaaacaactcacctgaggcctcacagccagtaagtgggttccctggtctgaatgtgtgtgctggaggatcctgtgggtcactcgcctggtagagccccaaggtggaggcataaatgggactggtgaatgacagaaggggcaaaaatgcactcatccattcactctgcaagtatctacggcacgtacgccagctcccaagcaggtttgcgggttgcacagcgggcgatgcaatctgatttaggcttttaaagggattgcaatcaagtggggccccactagcctcaaccctgtacctcccctcccctccacccccagcagtctccaaaggcctccaacaaccccagagtgggggccatgtatccaaagaaactccaagctgtatacggatcacactggttttccaggagcaaaaacagaaacaggcctgaggctggtcaaaattgaacctcctcctgctctgagcagcctggggggcagactaagcagagggctgtgcagacccacataaagagcctactgtgtgccaggcacttcacccgaggcacttcacaagcatgcttgggaatgaaacttccaactctttgggatgcaggtgaaacagttcctggttcagagaggtgaagcggcctgcctgaggcagcacagctcttctttacagatgtgcttccccacctctaccctgtctcacggccccccatgccagcctgacggttgtgtctgcctcagtcatgctccatttttccatcgggaccatcaagagggtgtttgtgtctaaggctgactgggtaactttggatgagcggtctctccgctctgagcctgtttcctcatctgtcaaatgggctctaacccactctgatctcccagggcggcagtaagtcttcagcatcaggcattttggggtgactcagtaaatggtagatcttgctaccagtggaacagccactaaggattctgcagtgagagcagagggccagctaagtggtactctcccagagactgtctgactcacgccaccccctccaccttggacacaggacgctgtggtttctgagccaggtacaatgactcctttcggtaagtgcagtggaagctgtacactgcccaggcaaagcgtccgggcagcgtaggcgggcgactcagatcccagccagtggacttagcccctgtttgctcctccgataactggggtgaccttggttaatattcaccagcagcctcccccgttgcccctctggatccactgcttaaatacggacgaggacagggccctgtctcctcagcttcaggcaccaccactgacctgggacagtgaatcgtaagtatgcctttcactgcgagaggttctggagaggcttctgagctccccatggcccaggcaggcagcaggtctggggcaggaggggggttgtggagtgggtatccgcctgctgaggtgcagggcagatggagaggctgcagctgagctcctattttcataataacagcagccatgagggttgtgtcctgtttcccagtcctgcccggtcccccctcggtacctcctggtggatacactggttcctgtaagcagaagtggatgagggtgtctaggtctgcagtcctggcaccccaggatgggggacaccagccaagatacagcaacagcaacaaagcgcagccatttctttctgtttgcacagctcctctgtctgtcgggggctcctgtctgttgtctcctataagcctcaccacctctcctactgcttgggcatgcatctttctccccttctatagatgaggaggttaaggtccagagaggggtggggaggaacgccggctcacattctccatcccctccagatatgaccaggaacagacctgtgccaggcctcagccttacatcaaaatgggcctccccatgcaccgtggacctctgggccctcctgtcccagtggaggacaggaagctgtgaggggcactgtcacccagggctcaagctggcattcctgaataatcgctctgcaccaggccacggctaagctcagtgcgtgattaagcctcataaccctccaaggcagttactagtgtgattcccattttacagatgaggaagatggggacagagaggtgaataactggccccaaatcacacaccatccataattcgggctcaggcacctggctccagtccccaaactcttgaacctggccctagtgtcactgtttctcttgggtctcaggcgctggatggggaacaggaaacctgggctggacttgaggcctctctgatgctcggtgacttcagacagttgctcaacctctctgttctcttgggcaaaacatgataacctttgacttctgtcccctcccctcaccccacccgaccttgatctctgaagtgttggaaggatttaatttttcctgcactgagttttggagacaggtcaaaaagatgaccaaggccaaggtggccagtttcctatagaacgcctctaaaagacctgcagcaatagcagcaagaactggtattctcgagaacttgctgcgcagcaggcacttcttggcattttatgtgtatttaatttcacaatagctctatgacaaagtccacctttctcatctccaggaaactgaggttcagagaggttaagtaacttgtccaaggtcacacagctaatagcaagttgacgtggagcaatctggcctcagagcctttaattttagccacagactgatgctcccctcttcatttagccaggctgcctctgaagttttctgattcaagacttctggcttcagctttgtacacagagatgattcaatgtcaggttttggagtgaaatctgtttaatcccagacaaaacatttaggattacatctcagttttgtaagcaagtagctctgtgatttttagtgagttatttaatgctctttggggctcaatttttctatctataaaatagggctaataatttgcaccttatagggtaagctttgaggacagattagatgatacggtgcctgtaaaacaccaggtgttagtaagtgtggcaatgatggtgacgctgaggctgatgtttgcttagcatagggttaggcagctggcaggcagtaaacagttggataatttaatggaaaatttgccaaactcagatgctgttcactgctgagcaggagccccttcctgctgaaatggtcctggggagtgcagcaggctctccgggaagaaatctaccatctctcgggcaggagctcaacctgtgtgcaggtacagggagggcttcctcacctggtgcccactcatgcattacgtcagttattcctcatccctgtccaaaggattcttttctccattgtacagctatgaagctagtgctcaaagaagtgaagtcatttaccccaggccccctgccagtaagtgacagggcctggtcacacttgggtttatttattgcccagttcaacaggttgtttgaccataggcgagattctcttccctgcaccctgccgggttgctcttggtcccttattttatgctcccgggtagaaatggtgtgagattaggcagggagtggctcgcttccctgtccctggccccgcaaagagtgctcccacctgccccgatcccagaaatgtcaccatgaagccttcattcttttggtttaaagcttggcctcagtgtccgtacaccatggggtacttggccagatggcgactttctcctctccagtcgccctcccaggcactagcttttaggagtgcagggtgctgcctctgatagaagggccaggagagagcaggttttggagtcctgatgttataaggaacagcttgggaggcataatgaacccaacatgatgcttgagaccaatgtcacagcccaattctgacattcatcatctgagatctgaggacacagctgtctcagttcatgatctgagtgctgggaaagccaagacttgttccagctttgtcactgacttgctgtatagcctcaacaaggccctgaccctctctgggcttcaaactcttcactgtgaaaggaggaaaccagagtaggtgatgtgacaccaggaaagatggatgggtgtgggggaatgtgctcctcccagctgtcaccccctcgccaccctccctgcaccagcctctccacctcctttgagcccagaattcccctgtctaggagggcacctgtctcatgcctagccatgggaattctccatctgttttgctacattgaacccagatgccattctaaccaagaatcctggctgggtgcaggggctctcgcctgtaaccccagcactttgggaggccaaggcaggcggatcaagaggtcaggagttcaagacctgcctggccaacacggtgaaacctcagctctactaaaaatacaaaaattagccaggcgtggtggcacacgcctgtaatcccagctatttgggaagctgagacagaagaatttcttgaacccgggaggtggaggtttcagtgagccgagatcacgccactgcactccaccctggcagataaagcgagactctgtctcaaaaaaaacccaaaaacctatgttagtgtacagagggccccagtgaagtcttctcccagccccactttgcacaactggggagagtgaggccccaggaccagaggattcttgctaaaggccaagtggatagtgatggccctgccagggctagaagccacaacctctggccctgaggccactcagcatatttagtgtccccaccctgcagaggcccaactccctcctgaccactgagccctgtaatgatgggggaatttccataagccatgaaggactgcacaaagttcagttgggaagtgaaagagaaattaaagggagatggaaatatacagcactaattttagcaccgtctttagttctaacaacactagctagctgaagaaaaatacaaacatgtattatgtaatgtgtggtctgttccatttggattacttagaggcacgagggccaggagaaaggtggtggagagaaaccagctttgcacttcatttgttgctttattggaaggaaacttttaaaagtccaagggggttgaagaatctcaatatttgttatttccagctttttttctccagtttttcatttcccaaattcaaggacacctttttctttgtattttgttaagatgatggttttggttttgtgactagtagttaacaatgtggctgccgggcatattctcctcagctaggacctcagttttcccatctgtgaagacggcaggttctacctagggggctgcaggctggtggtccgaagcctgggcatatctggagtagaaggatcactgtggggcagggcaggttctgtgttgctgtggatgacgttgactttgaccattgctcggcagagcctgctctcgctggttcagccacaggccccaccactccctattgtctcagccccgggtatgaaacatgtattcctcactggcctatcacctgaagcctttgaatttgcaacacctgccaacccctccctcaaaagagttgccctctcagatccttttgatgtaaggtttggtgttgagacttatttcactaaattctcatacataaacatcactttatgtatgaggcaaaatgaggaccagggagatgaatgacttgtcctggctcatacacctggaaagtgacagagtcagattagatcccaggtctatctgaagttaaaagaggtgtcttttcacttcccacctcctccatctactttaaagcagcacaaacccctgctttcaaggagagatgagcgtctctaaagcccctgacagcaagagcccagaactgggacaccattagtgacccagacggcaggtaagctgactgcaggagcatcagcctattcttgtgtctgggaccacagagcattgtggggacagccccgtctcttgggaaaaaaaccctaagggctgaggatccttgtgagtgttgggtgggaacagctcccaggaggtttaatcacagcccctccatgctctctagctgttgccattgtgcaagatgcatttcccttctgtgcagcagtttccctggccactaaatagtgggattagatagaagccctccaagggcttccagcttgacatgattcttgattctgatctggcccgattcctggataatcgtgggcaggcccattcctcttcttgtgcctcattttcttcttttgtaaaacaatggctgtaccatttgcatcttagggtcattgcagatgtaagtgttgctgtccagagcctgggtgcaggacctagatgtaggattctggttctgctacttcctcagtgacattgaatagctgacctaatctctctggctttggtttcttcatctgtaaaagaaggatattagcattagcacctcacgggattgttacaagaaagcaatgaattaacacatgtgagcacggagaacagtgcttggcatatggtaagcactacgtacattttgctattcttctgattctttcagtgttactgatgtcggcaagtacttggcacaggctggtttaataatccctaggcacttccacgtggtgtcaatccctgatcactgggagtcatcatgtgccttgactcggggcctggcccccccatctctgtcttgcaggacaatgccgtcttctgtctcgtggggcatcctcctgctggcaggcctgtgctgcctggtccctgtctccctggctgaggatccccagggagatgctgcccagaagacagatacatcccaccatgatcaggatcacccaaccttcaacaagatcacccccaacctggctgagttcgccttcagcctataccgccagctggcacaccagtccaacagcaccaatatcttcttctccccagtgagcatcgctacagcctttgcaatgctctccctggggaccaaggctgacactcacgatgaaatcctggagggcctgaatttcaacctcacggagattccggaggctcagatccatgaaggcttccaggaactcctccgtaccctcaaccagccagacagccagctccagctgaccaccggcaatggcctgttcctcagcgagggcctgaagctagtggataagtttttggaggatgttaaaaagttgtaccactcagaagccttcactgtcaacttcggggacaccgaagaggccaagaaacagatcaacgattacgtggagaagggtactcaagggaaaattgtggatttggtcaaggagcttgacagagacacagtttttgctctggtgaattacatcttctttaaaggtaaggttgctcaaccagcctgagctgttcccatagaaacaagcaaaaatattctcaaaccatcagttcttgaactctccttggcaatgcattatgggccatagcaatgcttttcagcgtggattcttcagttttctacacacaaacactaaaatgttttccatcattgagtaatttgaggaaataatagattaaactgtcaaaactactgacagctctgcagaacttttcagagcctttaatgtccttgtgtatactgtatatgtagaatatataatgcttagaactatagaacaaattgtaatacactgcataaagggatagtttcatggaacatactttacacgactctagtgtcccagaatcagtatcagttttgcaatctgaaagacctgggttcaaatcctgcctctaacacaattagcttttgacaaaaacaatgcattctacctctttgaggtgctaatttctcatcttagcatggacaaaataccattcttgctgtcaggtttttttaggattaaacaaatgacaaagactgtggggatggtgtgtggcatacagcaggtgatggactcttctgtatctcaggctgccttcctgcccctgaggggttaaaatgccagggtcctgggggccccagggcattctaagccagctcccactgtcccaggaaaacagcataggggaggggaggtgggaggcaaggccaggggctgcttcctccactctgaggctcccttgctcttgaggcaaaggagggcagtggagagcagccaggctgcagtcagcacagctaaagtcctggctctgctgtggccttagtgggggcccaggtccctctccagccccagtctcctccttctgtccaatgagaaagctgggatcaggggtccctgaggcccctgtccactctgcatgcctcgatggtgaagctctgttggtatggcagaggggaggctgctcaggcatctgcatttcccctgccaatctagaggatgaggaaagctctcaggaatagtaagcagaatgtttgccctggatgaataactgagctgccaattaacaaggggcagggagccttagacagaaggtaccaaatatgcctgatgctccaacattttatttgtaatatccaagacaccctcaaataaacatatgattccaataaaaatgcacagccacgatggcatctcttagcctgacatcgccacgatgtagaaattctgcatcttcctctagttttgaattatccccacacaatctttttcggcagcttggatggtcagtttcagcaccttttacagatgatgaagctgagcctcgagggatgtgtgtcgtcaagggggctcagggcttctcagggaggggactcatggtttctttattctgctacactcttccaaaccttcactcacccctggtgatgcccaccttcccctctctccaggcaaatgggagagaccctttgaagtcaaggacaccgaggaagaggacttccacgtggaccaggtgaccaccgtgaaggtgcctatgatgaagcgtttaggcatgtttaacatccagcactgtaagaagctgtccagctgggtgctgctgatgaaatacctgggcaatgccaccgccatcttcttcctgcctgatgaggggaaactacagcacctggaaaatgaactcacccacgatatcatcaccaagttcctggaaaatgaagacagaaggtgattccccaacctgagggtgaccaagaagctgcccacacctcttagccatgttgggactgaggcccatcaggactggccagagggctgaggagggtgaaccccacatccctgggtcactgctactctgtataaacttggcttccagaatgaggccaccactgagttcaggcagcgccatccatgctccatgaggaggacagtacccaggggtgaggaggtaaaggtctcgtccctggggacttcccactccagtgtggacactgtcccttcccaatatccagtgcccagggcagggacagcagcaccaccacacgttctggcagaaccaaaaaggaacagatgggcttcctggcaaaggcagcagtggagtgtggagttcaagggtagaatgtccctggggggacgggggaagagcctgtgtggcaaggcccagaaaagcaaggttcggaattggaacagccaggccatgttcgcagaaggcttgcgtttctctgtcactttatcggtgctgttagattgggtgtcctgtagtaagtgatacttaaacatgagccacacattagtgtatgtgtgtgcattcgtgattatgcccatgccctgctgatctagttcgttttgtacactgtaaaaccaagatgaaaatacaaaaggtgtcgggttcataataggaatcgaggctggaatttctctgttccatgccagcacctcctgaggtctctgctccaggggttgagaaagaacaaagaggctgagagggtaacggatcagagagcccagagccaagctgcccgctcacaccagaccctgctcagggtggcattgtctccccatggaaaaccagagaggagcactcagcctggtgtggtcactcttctcttatccactaaacggttgtcactgggcactgccaccagccccgtgtttctctgggtgtagggccctggggatgttacaggctgggggccaggtgacccaacactacagggcaagatgagacaggcttccaggacacctagaatatcagaggaggtggcatttcaagcttttgtgattcattcgatgttaacattctttgactcaatgtagaagagctaaaagtagaacaaaccaaagccgagttcccatcttagtgtgggtggaggacacaggagtaagtggcagaaataatcagaaaagaaaacacttgcactgtggtgggtcccagaagaacaagaggaatgctgtgccatgccttgaatttcttttctgcacgacaggtctgccagcttacatttacccaaactgtccattactggaacctatgatctgaagagcgtcctgggtcaactgggcatcactaaggtcttcagcaatggggctgacctctccggggtcacagaggaggcacccctgaagctctccaaggtgagatcaccctgacgaccttgttgcaccctggtatctgtagggaagaatgtgtgggggctgcagctctgtcctgaggctgaggaaggggccgagggaaacaaatgaagacccaggctgagctcctgaagatgcccgtgattcactgacacgggacgtggtcaaacagcaaagccaggcaggggactgctgtgcagctggcactttcggggcctcccttgaggttgtgtcactgaccctgaatttcaactttgcccaagaccttctagacattgggccttgatttatccatactgacacagaaaggtttgggctaagttgtttcaaaggaatttctgactccttcgatctgtgagatttggtgtctgaattaatgaatgatttcagctaaagatgacacttattttggaaaactaaaggcgaccaatgaacaactgcagttccatgaatggctgcattatcttggggtctgggcactgtgaaggtcactgccagggtccgtgtcctcaaggagcttcaagccgtgtactagaaaggagagagccctggaggcagacgtggagtgacgatgctcttccctgttctgagttgtgggtgcacctgagcagggggagaggcgcttgtcaggaagatggacagaggggagccagccccatcagccaaagccttgaggaggagcaaggcctatgtgacagggagggagaggatgtgcagggccagggccgtccagggggagtgagcgcttcctgggaggtgtccacgtgagccttgctcgaggcctgggatcagccttacaacgtgtctctgcttctctcccctccaggccgtgcataaggctgtgctgaccatcgacgagaaagggactgaagctgctggggccatgtttttagaggccatacccatgtctatcccccccgaggtcaagttcaacaaaccctttgtcttcttaatgattgaacaaaataccaagtctcccctcttcatgggaaaagtggtgaatcccacccaaaaataactgcctctcgctcctcaacccctcccctccatccctggccccctccctggatgacattaaagaagggttgagctggtccctgcctgcatgtgactgtaaatccctcccatgttttctctgagtctccctttgcctgctgaggctgtatgtgggctccaggtaacagtgctgtcttcgggccccctgaactgtgttcatggagcatctggctgggtaggcacatgctgggcttgaatccaggggggactgaatcctcagcttacggacctgggcccatctgtttctggagggctccagtcttccttgtcctgtcttggagtccccaagaaggaatcacaggggaggaaccagataccagccatgaccccaggctccaccaagcatcttcatgtccccctgctcatcccccactcccccccacccagagttgctcatcctgccagggctggctgtgcccaccccaaggctgccctcctgggggccccagaactgcctgatcgtgccgtggcccagttttgtggcatctgcagcaacacaagagagaggacaatgtcctcctcttgacccgctgtcacctaaccagactcgggccctgcacctctcaggcacttctggaaaatgactgaggcagattcttcctgaagcccattctccatggggcaacaaggacacctattctgtccttgtccttccatcgctgccccagaaagcctcacatatctccgtttagaatcaggtcccttctccccagatgaagaggagggtctctgctttgttttctctatctcctcctcagacttgaccaggcccagcaggccccagaagaccattaccctatatcccttctcctccctagtcacatggccataggcctgctgatggctcaggaaggccattgcaaggactcctcagctatgggagaggaagcacatcacccattgacccccgcaacccctccctttcctcctctgagtcccgactggggccacatgcagcctgacttctttgtgcctgttgctgtccctgcagtcttcagagggccaccgcagctccagtgccacggcaggaggctgttcctgaatagcccctgtggtaagggccaggagagtccttccatcctccaaggccctgctaaaggacacagcagccaggaagtcccctgggcccctagctgaaggacagcctgctccctccgtctctaccaggaatggccttgtcctatggaaggcactgccccatcccaaactaatctaggaatcactgtctaaccactcactgtcatgaatgtgtacttaaaggatgaggttgagtcataccaaatagtgatttcgatagttcaaaatggtgaaattagcaattctacatgattcagtctaatcaatggataccgactgtttcccacacaagtctcctgttctcttaagcttactcactgacagcctttcactctccacaaatacattaaagatatggccatcaccaagccccctaggatgacaccagacctgagagtctgaagacctggatccaagttctgacttttccccctgacagctgtgtgaccttcgtgaagtcgccaaacctctctgagccccagtcattgctagtaagacctgcctttgagttggtatgatgttcaagttagataacaaaatgtttatacccattagaacagagaataaatagaactacatttcttgca

SEQ ID NO: 8 - DNA, 81 bp, Homo sapiens
  source 1..81: mol_type = other DNA
ccttggccatgtaaaagtgcttacagtgcaggtagctttttgagatctactgcaatgtaagcacttcttacattaccatgg

SEQ ID NO: 9 - DNA, 85 bp, Homo sapiens
  source 1..85: mol_type = other DNA
tgcaggcctctgtgtgatatgtttgatatattaggttgttatttaatccaactatatatcaaacatattcctacagtgtcttgcc

SEQ ID NO: 10 - DNA, 3170 bp, Homo sapiens
  source 1..3170: mol_type = other DNA
aaacactctgtgtggctcctcggctttggtaagtgagctgccagcttccccaggcagaagcctgcctgccgattccttctttccttccctgacccaacttccttccaaatcctcctcctagaagccctccttggttggccctgcctactttaaagcttctttcacattttcttaggtcatgttcccctggggcctcctgccctcaaatgctttgctttttggcactctgtagatattctaaaaaatcattttgtacatgtgtgtgacaggccatctcccagttaagttgcagcctgtgctttctttttattttgcacttcccccactatttctgtgagtgcttagtaggaagtgtcaaagaagcttgacagcattttcttctaagtgtcccaactcttggttttccattacacagacagagtgcaagacgatgacttgcaaaatgtcgcagctggaacgcaacatagagaccatcatcaacaccttccaccaatactctgtgaagctggggcacccagacaccctgaaccagggggaattcaaagagctggtgcgaaaagatctgcaaaattttctcaaggtagggctggactctggcaggtctgacccagcctcaccgcagtttgggttgacaagggaggatgggagtatgggctacagcaatcaaggggaagatttgagctcctggagcccagccccaagacgcagcgagtgtcctgttatacagggcaggtgctcacagttacacaggacgacagggtcaagaaattgctcaattgaacacctgctatttgtcgggccctgttctgggcagagggatgtagtggtaaatggggagcccactattccagtggagggagacacacagtaaagttgttggccaataaagagcacagataaagccaaatgccaataagtgcctggaagaaaatgagatagagtgcgctgtgggcaatggggctgggtggggtggaggtgaccagttagggtacatgagaagggcctctttgaggaggtaacatttgagctgagccccgaatgttggggagggaagcccctgaggatgacacttggcacaaagctgaggagaccctaagcctcaggcgggaacttggggtggaagacttgggggcttttctaatcctaagggtctgcggtggaaaatgaatgcataaagagcacatggagagcacctgcacagcactcagggaactgggaggtttttcccccgctccaaaaatgattaggcagttctaagaaaaaggctgagcacttccaacagcctttttgttttcttttcaaatttggggaaagtcgggaaacagaggcctgcattaagaagggtggaacacatgggtctcagtctcagttccagtcccggagccagacatcctggggtaggtccccagccctcccagtgcccctccctccgccttggtaaggtggagaattgcagccttcagagttaggggccctgacagctctccataggtggaggcctcaggcaggcaggatgctgggtggggtaggcaagaaagggcccagcagagaggccgcatggcaaaactatcctccatgtgaccccctatgcccgcttcaccccccacctgacatcccccaccagaagcaaagcgatgctgtgggaaaggaagcagagcctcatggatgggctgcacaggagagtgctcgcattggctgggtaccccacaggttctgggaggggacttagcgaggtgactcagccagagggtggcagagctggaaccaaccagtgctctcttggaccccgcctgggtctgggtcttccacctcccctgatgtctctcctttttttttttttttttttttttttgagacagagtttcgctcttattgcccaggctggagtgcaacggcacaatctcggctcaccacaacctccacctcctgggttcaagcgattctcctgcttcagcctccagaatagctgggattacaggcatgcaccaccatgcctggctaattttgttattttttgtagagacaaggtttctccatgttggtcaggctggtctcgaactcttgaccttaggtgatctgcctgcctcggcctcccaaagtgctgggattacaagcatgagccaccctgtccgaccatctccccttttatactttatcacacccttgaggtcagcggagcacatactctgctctctgaccctccatctcccctgcccacacctagtttttctaggtgtttccccgttgtattggttgaaataagtttcactaattggtaacctccagagggaagggaagggagggcaggggaaggagtgaagtgcagaggggtagcagagtggaactggcctctaagtcagatctgaatttgcatgccctcaatagtcaagctgtgaaaactaatgaccctctctaggactggtttcaagtcttcctccaggaagataccattcctagctgttaaagttgttataaggaccaaatgaggtgacatttccaggcttactcatgccatgaccagggcaagaccctggaactcagcttcctcttctataaatagagaatcagcacccaagtcacagggtcatggagggaataaactggagagcgtttggtatgtgctcagtgtctgctccattgtgcgcactcagcctatggtcatttttaatttttaaatccagccccagggtgaggcttcccttgtacatttgccagctggtcatttactgtgctcccagtccccacctctggccacacccagctctcacagccttctctccccacccgcagaaggagaataagaatgaaaaggtcatagaacacatcatggaggacctggacacaaatgcagacaagcagctgagcttcgaggagttcatcatgctgatggcgaggctaacctgggcctcccacgagaagatgcacgagggtgacgagggccctggccaccaccataagccaggcctcggggagggcaccccctaagaccacagtggccaagatcacagtggccacggccacggccacagtcatggtggccacggccacagccactaatcaggaggccaggccaccctgcctctacccaaccagggccccggggcctgttatgtcaaactgtcttggctgtggggctaggggctggggccaaataaagtctcttcctccaa

SEQ ID NO: 11 - DNA, 2200 bp, Homo sapiens
  source 1..2200: mol_type = other DNA
cacaatggacaatggcaactgcccacacactcccatggaggggaaggggatgagtgcagggaaccccgaccccacccgggagacctgcaagcctgcagacactcccctcccgcccccactgaacccttgacccctgccctgcagcccccgcagcttgctgtttgcccactctatttgcccagccccagggacagagctgatccttgaactcttaagttccacattgccaggaccagtgagcagcaacagggccggggctgggcttatcagcctcccagcccagaccctggctgcagacataaataggccctgcaagagctggctgcttagagactgcgagaaggaggtgcgtcctgctgcctgccccggtcactctggctccccagctcaaggttcaggccttgccccaggccgggcctctgggtacctgaggtcttctcccgctctgtgcccttctcctcacctggctgcaatgagtgggggagcacggggcttctgcatgctgaaggcaccccactcagccaggcccttcttctcctccaggtcccccacggcccttcaggatgaaagctgcggtgctgaccttggccgtgctcttcctgacgggtaggtgtcccctaacctagggagccaaccatcggggggctttctccctaaatccccgtggcccaccctcctgggcagaggcagcaggtttctcactggccccctctcccccacctccaagcttggcctttcggctcagatctcagcccacagctggcctgatctgggtctcccctcccaccctcagggagccaggctcggcatttctggcagcaagatgaacccccccagagcccctgggatcgagtgaaggacctggccactgtgtacgtggatgtgctcaaagacagcggcagagactatgtgtcccagtttgaaggctccgccttgggaaaacagctaaagtaaggacccagcctggggttgagggcaggggtagggggcagaggcctgtgggatgatgttgaagccagactggccgagtcctcacctaatatctgatgagctgggccccacagatggtctggatggagaaactggaatgggatctccaggcagggtcacagcccatgtcccctgcaaaggacagaccagggctgcccgatgcgtgatcacagagccacattgtgcctgcaagtgtagcaagcccctttcccttcttcaccacctcctctgctcctgcccagcaagactgtgggctgtcttcggagaggagaatgcgctggaggcatagaagcgaggtccttcaagggcccactttggagaccaacgtaactgggcactagtcccagctctgtctcctttttagctcctctctgtgcctcggtccagctgcacaacggggcatggcctggcggggcaggggtgttggttgagagtgtactggaaatgctaggccactgcacctccgcggacaggtgtcacccagggctcacccctgataggctggggcgctgggaggccagccctcaacccttctgtctcaccctccagcctaaagctccttgacaactgggacagcgtgacctccaccttcagcaagctgcgcgaacagctcggccctgtgacccaggagttctgggataacctggaaaaggagacagagggcctgaggcaggagatgagcaaggatctggaggaggtgaaggccaaggtgcagccctacctggacgacttccagaagaagtggcaggaggagatggagctctaccgccagaaggtggagccgctgcgcgcagagctccaagagggcgcgcgccagaagctgcacgagctgcaagagaagctgagcccactgggcgaggagatgcgcgaccgcgcgcgcgcccatgtggacgcgctgcgcacgcatctggccccctacagcgacgagctgcgccagcgcttggccgcgcgccttgaggctctcaaggagaacggcggcgccagactggccgagtaccacgccaaggccaccgagcatctgagcacgctcagcgagaaggccaagcccgcgctcgaggacctccgccaaggcctgctgcccgtgctggagagcttcaaggtcagcttcctgagcgctctcgaggagtacactaagaagctcaacacccagtgaggcgcccgccgccgccccccttcccggtgctcagaataaacgtttccaaagtgggaa

SEQ ID NO: 12 - DNA, 8779 bp, Homo sapiens
  source 1..8779: mol_type = other DNA
cgcagcctgcagcccgagacttctgtaaaggactggggccccgcaactggcctctcctgccctcttaagcgcagcgccattttagcaacgcagaagcccggcgccgggaagcctcagctcgcctgaaggcaggtcccctctgacgcctccgggagcccaggtttcccagagtccttgggacgcagcgacgagttgtgctgctatcttagctgtccttataggctggccattccaggtggtggtatttagataaaaccactcaaactctgcagtttggtcttggggtttggaggaaagcttttatttttcttcctgctccggttcagaaggtctgaagctcatacctaaccaggcataacacagaatctgcaaaacaaaaacccctaaaaaagcagacccagagcagtgtaaacacttctgggtgtgtccctgactggctgcccaaggtctctgtgtcttcggagacaaagccattcgcttagttggtctactttaaaaggccacttgaactcgctttccatggcgatttgccttgtgagcactttcaggagagcctggaagctgaaaaacggtagaaaaatttccgtgcgggccgtggggggctggcggcaactggggggccgcagatcagagtgggccactggcagccaacggcccccggggctcaggcggggagcagctctgtggtgtgggattgaggcgttttccaagagtgggttttcacgtttctaagatttcccaagcagacagcccgtgctgctccgatttctcgaacaaaaaagcaaaacgtgtggctgtcttgggagcaagtcgcaggactgcaagcagttgggggagaaagtccgccattttgccacttctcaaccgtccctgcaaggctggggctcagttgcgtaatggaaagtaaagccctgaactatcacactttaatcttccttcaaaaggtggtaaactatacctactgtccctcaagagaacacaagaagtgctttaagaggtattttaaaagttccgggggttttgtgaggtgtttgatgacccgtttaaaatatgatttccatgtttcttttgtctaaagtttgcagctcaaatctttccacacgctagtaatttaagtatttctgcatgtgtagtttgcattcaagttccataagctgttaagaaaaatctagaaaagtaaaactagaacctatttttaaccgaagaactactttttgcctccctcacaaaggcggcggaaggtgatcgaattccggtgatgcgagttgttctccgtctataaatacgcctcgcccgagctgtgcggtaggcattgaggcagccagcgcaggggcttctgctgagggggcaggcggagcttgaggaaaccgcagataagtttttttctctttgaaagatagagattaatacaactacttaaaaaatatagtcaataggttactaagatattgcttagcgttaagtttttaacgtaattttaatagcttaagattttaagagaaaatatgaagacttagaagagtagcatgaggaaggaaaagataaaaggtttctaaaacatgacggaggttgagatgaagcttcttcatggagtaaaaaatgtatttaaaagaaaattgagagaaaggactacagagccccgaattaataccaatagaagggcaatgcttttagattaaaatgaaggtgacttaaacagcttaaagtttagtttaaaagttgtaggtgattaaaataatttgaaggcgatcttttaaaaagagattaaaccgaaggtgattaaaagaccttgaaatccatgacgcagggagaattgcgtcatttaaagcctagttaacgcatttactaaacgcagacgaaaatggaaagattaattgggagtggtaggatgaaacaatttggagaagatagaagtttgaagtggaaaactggaagacagaagtacgggaaggcgaagaaaagaatagagaagatagggaaattagaagataaaaacatacttttagaagaaaaaagataaatttaaacctgaaaagtaggaagcagaagaaaaaagacaagctaggaaacaaaaagctaagggcaaaatgtacaaacttagaagaaaattggaagatagaaacaagatagaaaatgaaaatattgtcaagagtttcagatagaaaatgaaaaacaagctaagacaagtattggagaagtatagaagatagaaaaatataaagccaaaaattggataaaatagcactgaaaaaatgaggaaattattggtaaccaatttattttaaaagcccatcaatttaatttctggtggtgcagaagttagaaggtaaagcttgagaagatgagggtgtttacgtagaccagaaccaatttagaagaatacttgaagctagaaggggaagttggttaaaaatcacatcaaaaagctactaaaaggactggtgtaatttaaaaaaaactaaggcagaaggcttttggaagagttagaagaatttggaaggccttaaatatagtagcttagtttgaaaaatgtgaaggactttcgtaacggaagtaattcaagatcaagagtaattaccaacttaatgtttttgcattggactttgagttaagattattttttaaatcctgaggactagcattaattgacagctgacccaggtgctacacagaagtggattcagtgaatctaggaagacagcagcagacaggattccaggaaccagtgtttgatgaagctaggactgaggagcaagcgagcaagcagcagttcgtggtgaagataggaaaagagtccaggagccagtgcgatttggtgaaggaagctaggaagaaggaaggagcgctaacgatttggtggtgaagctaggaaaaaggattccaggaaggagcgagtgcaatttggtgatgaaggtagcaggcggcttggcttggcaaccacacggaggaggcgagcaggcgttgtgcgtagaggatcctagaccagcatgccagtgtgccaaggccacagggaaagcgagtggttggtaaaaatccgtgaggtcggcaatatgttgtttttctggaacttacttatggtaaccttttatttattttctaatataatgggggagtttcgtactgaggtgtaaagggatttatatggggacgtaggccgatttccgggtgttgtaggtttctctttttcaggcttatactcatgaatcttgtctgaagcttttgagggcagactgccaagtcctggagaaatagtagatggcaagtttgtgggttttttttttttacacgaatttgaggaaaaccaaatgaatttgatagccaaattgagacaatttcagcaaatctgtaagcagtttgtatgtttagttggggtaatgaagtatttcagttttgtgaatagatgacctgtttttacttcctcaccctgaattcgttttgtaaatgtagagtttggatgtgtaactgaggcgggggggagttttcagtatttttttttgtgggggtgggggcaaaatatgttttcagttctttttcccttaggtctgtctagaatcctaaaggcaaatgactcaaggtgtaacagaaaacaagaaaatccaatatcaggataatcagaccaccacaggtttacagtttatagaaactagagcagttctcacgttgaggtctgtggaagagatgtccattggagaaatggctggtagttactcttttttccccccacccccttaatcagactttaaaagtgcttaaccccttaaacttgttattttttacttgaagcattttgggatggtcttaacagggaagagagagggtgggggagaaaatgtttttttctaagattttccacagatgctatagtactattgacaaactgggttagagaaggagtgtaccgctgtgctgttggcacgaacaccttcagggactggagctgcttttatccttggaagagtattcccagttgaagctgaaaagtacagcacagtgcagctttggttcatattcagtcatctcaggagaacttcagaagagcttgagtaggccaaatgttgaagttaagttttccaataatgtgacttcttaaaagttttattaaaggggaggggcaaatattggcaattagttggcagtggcctgttacggttgggattggtggggtgggtttaggtaattgtttagtttatgattgcagataaactcatgccagagaacttaaagtcttagaatggaaaaagtaaagaaatatcaacttccaagttggcaagtaactcccaatgatttagtttttttccccccagtttgaattgggaagctgggggaagttaaatatgagccactgggtgtaccagtgcattaatttgggcaaggaaagtgtcataatttgatactgtatctgttttccttcaaagtatagagcttttggggaaggaaagtattgaactgggggttggtctggcctactgggctgacattaactacaattatgggaaatgcaaaagttgtttggatatggtagtgtgtggttctcttttggaatttttttcaggtgatttaataataatttaaaactactatagaaactgcagagcaaaggaagtggcttaatgatcctgaagggatttcttctgatggtagcttttgtattatcaagtaagattctattttcagttgtgtgtaagcaagtttttttttagtgtaggagaaatacttttccattgtttaactgcaaaacaagatgttaaggtatgcttcaaaaattttgtaaattgtttattttaaacttatctgtttgtaaattgtaactgattaagaattgtgatagttcagcttgaatgtctcttagagggtgggcttttgttgatgagggaggggaaactttttttttttctatagacttttttcagataacatcttctgagtcataaccagcctggcagtatgatggcctagatgcagagaaaacagctccttggtgaattgataagtaaaggcagaaaagattatatgtcatacctccattggggaataagcataaccctgagattcttactactgatgagaacattatctgcatatgccaaaaaattttaagcaaatgaaagctaccaatttaaagttacggaatctaccattttaaagttaattgcttgtcaagctataaccacaaaaataatgaattgatgagaaatacaatgaagaggcaatgtccatctcaaaatactgcttttacaaaagcagaataaaagcgaaaagaaatgaaaatgttacactacattaatcctggaataaaagaagccgaaataaatgagagatgagttgggatcaagtggattgaggaggctgtgctgtgtgccaatgtttcgtttgcctcagacaggtatctcttcgttatcagaagagttgcttcatttcatctgggagcagaaaacagcaggcagctgttaacagataagtttaacttgcatctgcagtattgcatgttagggataagtgcttatttttaagagctgtggagttcttaaatatcaaccatggcactttctcctgaccccttccctaggggatttcaggattgagaaatttttccatcgagcctttttaaaattgtaggacttgttcctgtgggcttcagtgatgggatagtacacttcactcagaggcatttgcatctttaaataatttcttaaaagcctctaaagtgatcagtgccttgatgccaactaaggaaatttgtttagcattgaatctctgaaggctctatgaaaggaatagcatgatgtgctgttagaatcagatgttactgctaaaatttacatgttgtgatgtaaattgtgtagaaaaccattaaatcattcaaaataataaactatttttattagagaatgtatacttttagaaagctgtctccttatttaaataaaatagtgtttgtctgtagttcagtgttggggcaatcttgggggggattcttctctaatctttcagaaactttgtctgcgaacactctttaatggaccagatcaggatttgagcggaagaacgaatgtaactttaaggcaggaaagacaaattttattcttcataaagtgatgagcatataataattccaggcacatggcaatagaggccctctaaataaggaataaataacctcttagacaggtgggagattatgatcagagtaaaaggtaattacacattttatttccagaaagtcaggggtctataaattgacagtgattagagtaatactttttcacatttccaaagtttgcatgttaactttaaatgcttacaatcttagagtggtaggcaatgttttacactattgaccttatatagggaagggagggggtgcctgtggggttttaaagaattttcctttgcagaggcatttcatccttcatgaagccattcaggattttgaattgcatatgagtgcttggctcttccttctgttctagtgagtgtatgagaccttgcagtgagtttatcagcatactcaaaatttttttcctggaatttggagggatgggaggagggggtggggcttacttgttgtagctttttttttttttacagacttcacagagaatgcagttgtcttgacttcaggtctgtctgttctgttggcaagtaaatgcagtactgttctgatcccgctgctattagaatgcattgtgaaacgactggagtatgattaaaagttgtgttccccaatgcttggagtagtgattgttgaaggaaaaaatccagctgagtgataaaggctgagtgttgaggaaatttctgcagttttaagcagtcgtatttgtgattgaagctgagtacattttgctggtgtatttttaggtaaaatgctttttgttcatttctggtggtgggaggggactgaagcctttagtcttttccagatgcaaccttaaaatcagtgacaagaaacattccaaacaagcaacagtcttcaagaaattaaactggcaagtggaaatgtttaaacagttcagtgatctttagtgcattgtttatgtgtgggtttctctctcccctcccttggtcttaattcttacatgcaggaacactcagcagacacacgtatgcgaagggccagagaagccagacccagtaagaaaaaatagcctatttactttaaataaaccaaacattccattttaaatgtggggattgggaaccactagttctttcagatggtattcttcagactatagaaggagcttccagttgaattcaccagtggacaaaatgaggaaaacaggtgaacaagctttttctgtatttacatacaaagtcagatcagttatgggacaatagtattgaatagatttcagctttatgctggagtaactggcatgtgagcaaactgtgttggcgtgggggtggaggggtgaggtgggcgctaagcctttttttaagatttttcaggtacccctcactaaaggcaccgaaggcttaaagtaggacaaccatggagccttcctgtggcaggagagacaacaaagcgctattatcctaaggtcaagagaagtgtcagcctcacctgatttttattagtaatgaggacttgcctcaactccctctttctggagtgaagcatccgaaggaatgcttgaagtacccctgggcttctcttaacatttaagcaagctgtttttatagcagctcttaataataaagcccaaatctcaagcggtgcttgaaggggagggaaagggggaaagcgggcaaccacttttccctagcttttccagaagcctgttaaaagcaaggtctccccacaagcaacttctctgccacatcgccaccccgtgccttttgatctagcacagacccttcacccctcacctcgatgcagccagtagcttggatccttgtgggcatgatccataatcggtttcaaggtaacgatggtgtcgaggtctttggtgggttgaactatgttagaaaaggccattaatttgcctgcaaattgttaacagaagggtattaaaaccacagctaagtagctctattataatacttatccagtgactaaaaccaacttaaaccagtaagtggagaaataacatgttcaagaactgtaatgctgggtgggaacatgtaacttgtagactggagaagataggcatttgagtggctgagagggcttttgggtgggaatgcaaaaattctctgctaagactttttcaggtgaacataacagacttggccaagctagcatcttagcggaagctgatctccaatgctcttcagtagggtcatgaaggtttttcttttcctgagaaaacaacacgtattgttttctcaggttttgctttttggcctttttctagcttaaaaaaaaaaaaagcaaaagatgctggtggttggcactcctggtttccaggacggggttcaaatccctgcggcgtctttgctttgactactaatctgtcttcaggactctttctgtatttctccttttctctgcaggtgctagttcttggagttttggggaggtgggaggtaacagcacaatatctttgaactatatacatccttgatgtataatttgtcaggagcttgacttgattgtatattcatatttacacgagaacctaatataactgccttgtctttttcaggtaatagcctgcagctggtgttttgagaagccctactgctgaaaacttaacaattttgtgtaataaaaatggagaagctctaaattgttgtggttcttttgtgaataaaaaaatcttgattggggaaaaaa

SEQ ID NO: 13 - DNA, 9609 bp, Homo sapiens
  source 1..9609: mol_type = other DNA
gcagttactgagaactcataagacgaagctaaaatccctcttcggatccacagtcaaccgccctgaacacatcctgcaaaaagcccagagaaaggtaatatgaatgaaataattttgggggactttaattgaggagtaaaatatttgagaatatgaggaagattccaaagtctctgcatataccttaataagaactgagacaggcttttactcattctcttttcagcacttatgattgaattagaaggaagtctgtaaaatttggctgtgatcatagggtaagatgttatctaacagaagccagaaacccaatgtctcctgctgagatgcttgagtgcctgtcaggatctaaaaattttcctcaagaattactgtatgtcattggaaagacgttcttttgagtggcttccaggagccagacagagggcaagtagacattatgatattgttttattatccatttttaagtgatgtatagctatatcttcaagctggcccatgataaagtggttcacttgttcagctgaatgactatagcttctgattatcttttgaatagatgttctcatgcagacttgaatagtagcatggaatttcttgaatgtcgttgttttcatttttcttctttaataaaatgctacaaaaatcaaagttggtagtatttctctagctattattcatgaatttgcaatgataagtcacttgcccaagtctaattgattagttccaatgagtttctggaaacttttttgcagctaaccttggttatcttagcattagcattaattggtggctgattgggaaatagacactagaaaataaaagaccttttttgtccctccttattagcgttgaagaataggctatgggcacgtgtgaagaactatgggctgacactatatgggtcccttaggaatgcagaagctccctttcatctctgtagatattttgtttcttaagctcttcaatctttttcccagtcaaaagtcagatattttgctttagaaaaggaatcttttaaagtttctgaaaatatcttttaaataattacttgacttaataccaattcaattattcataatattggtcaaccaaattgcatgtaatacattgctatattcttgaattatttaaaaaagacaagagtggtcatcatttataaaaggttcgtggtttttcatgttaatttcaactttggttttcttaagtttattattttttttgcagtaagagtcattgaaattttaagtgagtcatattccttaccatttcctgctgaaaagggtagtgtgtgagaaaaatgttagaaaagcaattaattatgttccagagcagattttcagttgcagtgtacatttctttttaatgtgagacccaaatttacatgaaaactcaaagtaagagctgggtaacagaaatggctaacttagaaggtaatgtacgtcttgcttaaaagcacatcaaagtaatctactttctcaaagagaaaatttacaggagtgaacttacatttcttttgagaacagcatggttcatagcaccaaacttcatttttacaggttgtgaatcctagagtagtttgctatcaacttctgatctttgcacattctggatttggcatataatgttacagcagtgccattgtaatgttgcacaaagtagtctagcaatttcttggttcaccaggcttagagataacattgtagaaatgatccagcatctttaacactctgtggtttaaggtggggcacttaggggtagaatcaataacaatgttagaaatcaaattagacaagataactgaaacagcatgatccatgtgtgactccaagttataaaggaggacatggattaatggtatacttctaggctataggggtagtacaagtggaaggacaccatcttagcatcagatcactttctgagcaactttggcaaatcttttaaattctctaatgtgtagttttttaatatatgacacaggtgtaaagaaaataaagcaagtgaatgtatgtgaaagccaatgctgactgggcacgggggctcacgcctgaaattctagcactttgggaggcagagccggggatatcacttgagcccaggagttgaagatcagcctgggcaacatagagaaaccctgtctctacaaacaaaacaaaacaaaaaaacaaacacaaaaaaccactcccaaattagccgggcttgctggcacactcctgttgtcccagttacccgggaggctaagatgggaggatcacctgagcttgggaagttgagactgtaatgagccgtgatagtggcactacactccagcctgatccacagagtgagaccatgtctcaaaaaaaaaaaaaaaaaaaaaaagaaagctaatgctttttcccctttccctgttcccctgttgttccccactgcagacagtccttatagcttgatcagtttaaaatacctgaacttgctctcttttcttttcttttttcttttctctctctctttctttcttttcctctcctttcccctcttcccctctcctctcctctcctcttcttttctttttctttctttctctctctctctctctcttttttgttttcaagacggggtttctcactgtctcccaggctggagtacagtggctcgatcccagttcactgcagcctcattcactcaggctccagtgatcctcccacctcggcttctaagagatgggaagcaggaactgccaggtcagttaagggatatacctactacttgcccagtgtcactactgctatattcctgatctaagcagtcaagggcctatgtagatgaaatggggtacaaagataaaaatacaaagacagacataccactgtttgacgtgggagtgacaaggtcacactgcaaataaatgtaggctgaggggtatttttgtggccatttttggaaagtacaatctgccatagcagtaaacacaggggcaatgaacaaggggcttcactttgcagctcctctgctctgtttttattaccaaaaaaaaaaatccttttaaagtaagatgcctagacaacatagtgagatgcccacttcttttcttttctttctttctttctttttgagacggagtctctctgttgcccagggtagagtgcagtggcgcaatctcggctcactgccgcttccacctctcgagatcccatttctaatttaaataaaaagaaagaaagtttctttgtggatgaagagatagacgtgtacataactggttagactgtggggcatcatctaagaattataagccaagtgataagtgagtgcagtggagaaagatatttattttgtctttggggttgggtgaaaacttcacagtgaatctggctgttgaacagctccttaaaagactctgaagtagatgaactgaaaagggagagaaagaaggccaagttgagaaaactcatgttttcttggacacatattatcttgatgtggtgggtgatgggatataagggtatgttggtgtgtattgcaggttagtctgaggttgtgtgtacagggcctttgaagttcggaaaatactcatgtgaaataccaaaagaagctgagattagtaaatctgactttagattgagcatatttttgcaaaatagcataaatcctagcagaatttaatttctccccctgattcttaatattttcttttgaattttaaaacagaaaaacctgagggtgattaggatgataaaaatatttattaaaatgctttcaaaatcacctagaatttgaaggctattctgtttttacttggttaatgtcatctcttttcaaaatacaggcaaagaaaggtaatagtttctgctacagcaatagtgatttttgtttcactttttcaatcttcttttcactttattataaaggcaattctaaaatgcgcattgacttcatgctttcacattctcaaatcttattataaatgtttctctctgaattaattctgatatagttgttcactgcataatggctgaattttcataatatatgagctgcaatattaaggcacaaacatgatactagtttaaaaaggaaactagttttaattctgaacatttccttatggctttgtgtattctcaaacttactgatctcagaacctgtttacactcttaaaaattattgaagagcccaggctggtcatggtggctcacgcctgtaatcccagcactttgggaggccgaggcaggtggatcacgaggtcaggagtttgagaccagcctggccaatatgctgaaaccccgtctctactaaaaatacaaaaaaaaaaaaaaattagccaagcgtggtggcatgtgcctgtagtcccagctattcgggaggctgaggcaggagaattgcttgaacccaggaggtggaggttgcagtgagccaagactgcatgactgcattccatcctggacaatagagggagactcaatctcaaaaaaacaaaaaaaaaattattgaagagcccaaagagcttctattcatgagtttatatccattaatatttaatggcttagtgattatgctaaagtttaaaaatatttattcatttagaaaaatccatcatatgttaacacatataacatatatttattttttaaaaatgacaattttcaaaaaaaaattagtgatgagtggcattgttttacccttttgcaaaactcttcatcgtctggcctaacagaacatagctaaattctcatgtgctttttcattcaatctgttgtaaaattacatgtcatgtagcctctagaaaatttctctgaacacccaagaggatgaagaggaaaaaaagacaaacaacattttagtattattatgaaaatcattttaaccccacagatccactgaaaatctttggggttcccagatcacactttgagaaccactgacttagaacaatatttattcagtgttaattatgagtgaagataaatagaactcaaaattacttacatataaatatatatattaggtagaaataatgacataggtttgttttagccttcatacttacacaatctgaatttctatacaggttgagtatcctttatctgaaatgctgaggatgaaaggtgttttagattttaattttttttggatattggaatatttgcatacacatagtgagatatcttggggatgagacccatgtctaaacataaaattcatttgtttcatatacacatagcctgaaggtaattttatatactattttaaatattttgtgcataaacaaagtttctgttaagtacttatatgtggaaatttccacttgtgtaatcatgttggtgcgcaaaatgtttcagattgtgggccatttcagatttcagatgttcagaatagatatactcaacatgtgttataaacttagttctgctgtctgataaattattcctaagaagtattatgggttaatataaacatctagcagaaactcagccctattatgtcagtctacatgaaaaataaccataagttttgactcatatgtacctttaaacctcattctgaatttttttaaaaaaacttttattttgaataattgcagatttagaggaagttgcaaaaaatgtacagagaagtcctgtatatccttcagcttgttccctcattgaaaattatcttgtataactatagtacaaggtgaatactagagaactgacattgctgccgcctatacagcttattcagatttaagacacacacacacacacataatactagtgctctgttatgcagttttatcccatgtgtagattagtgtgactaacatccctatcaacatgcggctgtcccatcaccacagctcccttgtgctatccctttagagccatactcaccctcatacacttctttcccagtgctaactctttgaaaccattaatctattctctatctctataattttgttatttccacagtgttatataaatggaatcatatagtattcagcctgcattcagcacaattctcttgagatccattcaagctgctgtgtgtatcaatagtgtgttcatttttttgttgctggacagtattccatggtatggctataccatcatttgtatgaccattcaccttctgatggacatttgaaatgtttccaatttttggctactctaaacaaagtttctatgaatatttatatataagttttgtgtgaacatagtcttcatttctctgagataaatgcccaaaagtgcaactgttggggcatatggtaagtacatgtttagttttatcagaaactgccaaagtatttcccagagtggctgtaccattttgtattcccactagaccagcaatgcctgagttatctggattctctgcatccatgccagtatttggtgttattttttattttagccattctgatagatatgtaatatgtcattgtagttttaatttgcatttccttaatggctgataatgttgaatactttgtgtttatcctccatcaaatgattgtatattttatatctcatatataagtttatatatattttcttaggtattatctagtttaagttccatgttttacaaataaggacattgaggcttcttaacaggatgacagataatttaaaatttaaattttaaagaatttaaaaagagaattttttgtaattattattaaaccaatttctacagttaatgtgagaaatgggaagattcagttatctatctctttcctaaggagaactttttttaaaaaaaattacatggttttagtatatgttgggagctaaaagcagggaggtcaagacactgatgactattattaatagtaatgttgaaactactggttgttgttatgactggtaagccaattttagattaactgttttttgtttttttttttttgccatgtctgtctgcaggagcgccatggattactacagaaaatatgcagctatctttctggtcacattgtcggtgtttctgcatgttctccattccgctcctgatgtgcagggtgcgtgaccaaatttgtggttcaagtaataaggacaacacacatttctagatgtacatcaataactccattaattacatttctaccaccttttcaaaagtaataagtctttgctgctggattcatatctaggcacttgtagattgtgaacataaaattaaattaggttcagaaaatgtgcagtgaaaatgatatcttacacaaccatttatgcagcagcctatacattttcatcggaaatagattcctttttattcttgagtcttacaagaagaaaatgctccttattcagttagctcagttattttttacatttctcccggcagatttgagattttaacattgcctttgtagatgaattttcacatcagttaacaagtgagaaaaacaaaaccattttatacagtaaatttgttttgctgtattgtctgaaaaatctcatatagtagctggtataattccttctgctttgaaattgtgagctactattggttatggtttttctctatataagtggtaatattttaatccaggtcccaagtgcaggcgcgtgatctaatatcaggctctctacactcaccaagctttcttaattctgacatatttctctctgtcaatatttggagttactgtgggaaaaacaatagcagattctaaagggaaaaatatttttcctctgtgcaaaattctcttttcagatgaacatgatgttttcatctgtcaagttttgtgtttcctctaggcatactgttagcattgggatagagaatccatgcttgaagagagactacaactgagattttctatgcatatctgtaaaaaatgtttgtttttaagttttatttcccatgaacattaatcagtataaatattaaatagatattatagatgaagattaacatataaccaaaaagcacttacttagtttcctttcatttttgatgaaaaaataatattcactatcccataataaggaagcattcacagtttcttttctttgttgccttgccttgtcttgccttgccttttcttttgagacagagtctcgttctatcacccaggctggagtgcaatcgtgtgatctcagcttactgcaacctccgccttccgggttctagtgattcttctgcctcagccttctgagtagctggtattacaggcacctgccaccatgcccagcgaaatttttgtatttttagtagagatggggtttcaccatgttggccaggctggtctcgaattcctaacctctggtgatccacctgcctcagcctcccaaagtgctcggattacaggcgtgagccaccacattttttcttatttttttgagtcagggtctcactttgtcacccaggctggagtgcagtggcatgatctcggctcactgtagcctcgacctcccagcttcaagcgattcttctgccccagaccctcaagcagctgggactacaggtgtgcaccatcacgtctggctaatttttgttgttgttgtattttttgtagagacagggtttcaccatgttgcccaggctgctctcaaactcctgagctcaagcaatccacccactaaggcctcccaaagtgctaggattacaggcgtgagctactgtgctggcctcatagattctttttgagtcttttttggatattttactctgcctttttttttccctgatagattgcccagaatgcacgctacaggaaaacccattcttctcccagccgggtgccccaatacttcagtgcatgggctgctgcttctctagagcatatcccactccactaaggtccaagaagacgatgttggtccaaaagaacgtcacctcagagtccacttgctgtgtagctaaatcatataacagggtaagaacctcaagatccccagaagctttctaacagcccaatcagagaaatgttcatagagcccacccatggaatttaatgccaaaggtgtctaatgacccagcctctgtcgagcatttgtacaggtggggaatacatttctacccattaattaaaagagtcaattgtcttgtgggtatagactggatttattcagaatgaggagaataggggtagaggtgacaaggggcaggttgggagaaagtacagcttacttgtgctaaaaatatttcctaaaaaggagactgtgcaaatgtagtatgcatctacttatttcagcagaatgcaaacaattttatgtaatattcttcaattttgtctctatctatctatctatcatctaatctataatatgtttttttttccttcccctttaggtcacagtaatggggggtttcaaagtggagaaccacacggcgtgccactgcagtacttgttattatcacaaatcttaaatgttttaccaagtgctgtcttgatgactgctgattttctggaatggaaaattaagttgtttagtgtttatggctttgtgagataaaactctccttttccttaccataccactttgacacgcttcaaggatatactgcagctttactgccttcctccttatcctacagtacaatcagcagtctagttcttttcatttggaatgaatacagcatttagcttgttccactgcaaataaagccttttaaatcatcattcaa

SEQ ID NO: 14 - DNA, 16352 bp, Homo sapiens
  source 1..16352: mol_type = other DNA
gtaggaatcgcagcgccagcggttgcaaggtaaggccccggcgcgctccttcctccttctctgctggtctttcttggcaggccacagggccccacacaactctggatcccggggaaactgagtcaggagggatgcagggcggatggcttagttctggactatgatagctttgtaccgagttctagccagatagaaggttaccgggagctggggagcgttggatttgctgctgggctgtgccggtgcccagaaggcaggaccttgcagaaccagccaggtccctgggagactgtcagacccaccaacctggtggcattcgcagagctgagatgcattggaaattgccttgggcacatccccaaagatcaggatgtcccaccccagtctgaaggagataaagttgggggtaggagagacgcagatgcaagtgatcagtctcagtcccagacattgccttgctctgcgggtaggaattcaggattcattttccagggaagttcctgacctctgaatgagaggggctgtgtaaggccaatgcctgggaggaaggcaaggatgagtagaggtggggggaaacaagtgtcaggaagactcaaaatcttccagagaaattgtgcagggtcttaccagatctgtcctcaaagccatgcaaattgccttctttgcaatgcatacaatgaggtgtctctgggggtcagaactggttattagggaacttctagccaggactgctaaatacgcgctgttggcccaccaggctcacctatagccttccttcagtctgggcttggtttggatttcactgtgggtgccatcgcctttacactcctgtttctatagtttaaagatagtggtgctttgggaaagtgactccttaaatacagttaggtccaagtgagacaagtggcctggctgtcatttcagaatagcagcttccaagaggtgattaatttctgttggaagggtgatctttggggaggtgggtgaagagcagagacttggtggtaccgttccaggagcacaggctctcttcctttgcagtgcagaatgacctctggcagccggagttgtgtttgttctgtaggattctgaggtgggccatgggcagctggaactggggaattttgccaatctctttcatattaggattgtctgcagaaccagatatggaggcttctagcaacgtgagtgctcctgttctaatgcccttagaaacaagaaggccacactgatcatttctctcacttaggcagggagacaaggcaagagagaaacagtggatgcttttaggttctttcccttcccaagcagttgtggacattgggctgaggggaacatttccacattggctaaaggagcgtcctcctcatattttgtacattttatacccaaaataactcttcttggtatttggggaaatattttcctccccgtccattccaggaaatggctccaagtgccaaggacagagccagggaagttgcaatgaattcctgcccgtcagccccaggcagatgccttgcacgtctgagtggcccatgcagagcgtggaggtggccgccacggaacctgggtcaatgtcccacccccgcttagatgccaccaggggcgtgggagccaaggagagaagaggggctccaggaaggtagagtccttgtgtcttgtgcatctgtgaacagcactggtatgatttaaaggaaaattgagccaaattttccggcagtcagttaccccatccccaccggggtaggagtctggcagccgcagctccattctggccagtcggcagagagccttgaaattcttctttgtccacacagttgtctcagagaaacagagaggttgtttctgcttaaaaacaacacacttggtgtctgggcccacagactcctttgcacttattccacgtgtgacagccaatgtgcctcgttgcttagcagacagcatgttaccgtctttcctgctcagtttgttagctctatggaatggaatttataatcaatgcccataccaacatttcactaatatcataggagatttagtctccatctgggtgtacattacatttgctctggggtgctccaggctggggggttgccaaggaagagaagagaaaccgcagagaagacgggagggcagggcaggggtctctgagaaggggaggggtcccagagtgcaggagcaggagccaggctcatgaaaggggccacgggcgggagtatccagggacggcagtcaagatggagcacagcttaggaagctgaagggaatcctggcccacctgggtgctagagggcacataggaagtgcaggaagcagaccaaggtccccaagagagggagacctggacgctgaagcattttctgtctttattaagacaactccgtaagaattcctgctgggccaaagtgaattctaggatgcgactttaagatgggagcaagcgaaccattgaggaggcaggttaccctagttagccaatgcagatcgagaatgggaaatctttcatttattcatgcaacagatatttaacgaagccctgccgtgttccaggcctgtgatagatgctggaacaggtacagagatacaggtgtcattaattgatcagggcaacctctccttctgagtcttgctggagcttcagatgcccctcacacagagctcgagggagcctcaacaattgatcagaagtcaggcaccatggctcacgcatataatcccagcactttgggaggccaaggcaggtggatcactggagcccaggagttccagatcagctggggcaacatggcaaaaccccatctctattaaaaaaaaaaaaagtaactggatgtgatggtacacacctgtagtcccagctacttgggaggctgagaggtgggagaattgcttgagcccgggaagtcgggggtccagtgagccttgatcacaccactgcactccagcctgagtgacagagcaagaccctgacacacacacacacacacacacacacacacacacagattagagctgaaacaggagtagaaacctatctgtatctctgatgagatcagatctttctgatgaacagaaagaatgtaacccctgtactcacaccctctctgctggttacatatgttaacacgatttctcaaatgaggcttttggttgcaaataagagaaaatcactcacgctggccctgtgtttttcaaattgtttattgtgatcaacatttgaaaaaagagccgagactctcaagagtgcattacccacggtaagggtgaattttacttcttgacacttatttctcttacatgtatctatctgtctcaaatgaaaaatatatttagaaagttgaaagctatccaagtgagtataagaaaagagtatctcaccctgaaggctaaggacagggagggccaccaggcctcacgaggacccaggaaccacaaagaaggctaggaaggagcacaggcggtgaccatactctggctcagtggctatgtgggctctggtctctctcagctgttccatgcatatgaggccaaatgtggctaccctagagcttctgagccctcaacagagatgaactggactctctgcagccccactctaaattcctaagagagaagttgattgacccaatcagggtcaggagaaggaagggaggaggaaagggaggagagaagagcctcttcgtctcttgcctaccactggccaggcaattgtagccaagggggctggagtgtaaatgcaaacatagccatcaagggttgtgtatgtgtgtgtgtgtgtctgtgtgtgtgtatgtgtgtctcttgggtaggttagatctcccaggaggtccctactaaacagacttaagcccgcaaaattttagctctccagcctcacacactccacccctctaccatattgaatcttcccaaaccaactatggctttccctaactccggagcttggcctggaatgccctgcttcccctctttcccctggggaacgcctgtccttcaggcctcagttcacacactgcctcccttgcaaagctctcctcccatccccggagtccctcttcccctttgttctttgggttctatgcttcttccctcataactcccaccaggttgtgttaaaatgagttgttcaaggtcctgtctgttccactagattctgagcaacttggagaacgaagatccaaacttcgctgcctttatttcctcctttgttcttttctcatccccaagtcccttccaacttggagttatgaagaaaggaaggaaggaagggtgggagggaagaacaggaggggatcccacaggagaatgtgtatagggagaggactcagactagctaaagcttttccctcataattaatagcaaataccatgttacctgaatttaattcacagtagcatacaaaagactcgctttgttctccccattgatgtcatcagagggctgtgggcaggcctaatcttggctcaggaggccctccagcctggatctaaagagcagcagatgggccaggctcggtggctcatgcctgtaatcccagcattttgggaggccgaggcgggtggatcacgaggtcaggagtttgagaccagcctggccaagatggtgaagcctcgtctctactaaaaatacaaaaattagccaggtgcggtggtgggcgcctgtatttccagctacccgggaggctgaggaggctgaggcaggagaatcgcttgaacccgggaggcggaggttgcagtgagccgaggtcacgccactgcactctagcctgggcaacagagcaagactccgtcaaaaaaaaaataaaaaaataaaaaaataaaaaaaataaagaggagcacacatctctgcccatcctaactcccactttgacattgaggtccccaggatggagggtctgcctccatctgccttgtcccctgcaatggtgggaaggtgatggagctcaagtctagaggccaccagcttcttagggaggtaggaggtggagggtggggtgcgggccctgcacacaactgccaagtgaggatgggggtggggtccacctgaggataagtaacagtgaggctggtgcagaggacccaggtggaggtagacagcagaatttgtggtggggtggatggcacattatataagcctctcttgctgccctgtttactgagattgtttcattatcttttttggcttttgtttttaagagatggggtcttgctgtgtcacacaggctggagtgcactgtgtgatcatacctcactgcagcctcgacatcctgggctcaggcaaacctcccaccttggcctcccaagtagctgggaccacaagcgtttgccaccacactcagctatttttatttttatttttattttttttagagatggggtcttgctgtgtcgcccaggctggtcttgaactcctgggctcaagcgatcctcctgccttggcctcccaaagccctgggattataggctgagccaccacacccagccacatttcatctgtgcagctccaggggctccacattctactcttctcatttcttctccagggtacccatggcaagggatgagggtagaagatggggcagccaggccttgattaaaggagaaggaaggcagcctgtggagagggcagcccagggagtgcagagagaagtgggccatgagggagacagcagagtgcaggctgcgtcccaaatgagcatacagcccactgtgagcccaccatcttcctagagacccctctcctctccaggagctgcttcagtagcactcagaggaaagaatgatgctgtatcaacatttcagcagctcatcttttaactctaagaaaatggcagctcctaaatgttcaaaactgctttggaaacttctggagagaggttttgcagctcaggcagacagctgatcgcggcctttcttccaccccaacccatgctctccccatgctctcctgccacagctgcagcgggcccctgggtcctacatttgcagccctttgtctctgagctcagacttccaattccaagcggcagctgggcaggctcaccagcatgtccagccagtactaggacatcagcaggagcccaaccacctctttccaaaatctctcctcatgtctctcctagtttccatctccatccttctagtcagccaggctgaaaacatttgctcctcagggtgcagaagggaaagctttgcctcccttcctggtgctcactgcccctgcgattccagcccaagccctccccggctcctcaccctggtgtcagctggaagccaccatctcctaaacccacctgtgttcttccacctctgccagggctgccctctcctccaccttcacaaactcaattcctacccattctcaggtcccttatcaaatgccatctcctccatgatgcctccctgattcccctgctggaaataatggtgataacagctaaggcattggggttggctacgtgccaggcaaggagttggcactttacatgctttatctcatttcagccacataacatcgacaggtggcattatgattcatatcatccccatctgatagccaggaaaactgagtcccagagaggttagccactttcctagggccctgtgctctgactcaagcatagctctgaggaactctagcattcatcagtttaagcaccatgactttctttgctgagtcacccaaggcatttcttcatttaaatgttcttccttggccaggcgcagtggctcaggcccaatgcggtggctcacgcctgtaatctcaacactttgggaggccgaggtgggcagataatctgaggtcaggagttcaagaccagcctggccaacatggtgaaaccccatctctactaaaaatacaaaaaaatgaggctgggcgtgatgactcacacctgtaatcccagcactttgggaggccaaggcaggtggattacatgaggtcaggagttcgagaccagcctggccaacatggtgaaatcctatctctattaaaaatacaaaaaattagccaggcatggtggcaggcacctgtaatcccagctacttgggaggctgaggcaggaaaatggcttgaacccgggaggtggaggttgcagtgagccaaggttgcaccattgcactccagcctgggcaaaaagagggaaacatcgtctaaaaaagaaaaaaaaaaaattagccaggctgggtggtgcatgcccgtaattccagctactcaggaggatgaagcaagagaattgcttgaacccaggaggcagagattacagtgagctgagatcacaacactgcactccagcctaggtaaagaacaagactccatctcaaaaataaataaataaaaataaatgttcttccttgcaatgaagttaaatatgtaaattctcaaaccagttgcttaagggcacagttttgttctttacctatatttttaacaaatattttatgtaagtagttgacaaaatcaaatactgtgtacactaccgaggcttccctgggaaagccatcagcctctgccccatcccttcccactcctgattccactttcctgtgtttccatatctttttcatgtctgtttctggcccacagtgggcgatcaatacatgttagccaccaaccatcaaacctatattgagtaattatggtatgtcaggcactatgctcaatgaaattgtattaggcttgtacaaaagtaattgtggtttttaagagtaatggcaaaaacggcagttactttcgcaccaactatttgctgccttgaattattcctcctctcctcatccctaaaccctgctcctcccagccattcttcctccccttcttgggccatggccaggccccacccaggtactaagactcaggtgaaccaaggaagacttaatgcccactcttttctgatgcccatgttggcatgtgttaagtcggttagcattaagtttggctgcatttagcagagacccaaaagaacagtgccttttaaaaggcagaggttatgtctctcacacacacccagcacaagtccaagaccagcatggcatctcagctccatcaacctcaggaaccgagctcctgcagctccctgccctgcagttgataaggtgaggtctttgtcctcctggttcaagatggtgctagaatgttggctaccatatctatagtccaggcatcagaatggagcaagggatgaaaaaggaagagatgaaggcacacgacaggttcctgagagctggcacaggacacttctgcttatatttcactggccagaacttagtcacatggtcacacctagttgggagactctgagaagtaaagtatttattctagatggccatatccctacctaagacttggagttttctatgactggggaagaacggaagacaagatattgggaaagactagcagcctctactaaaagggtgatctgtgttgatgtgcgtgtgtgtgtgatgtttgtatgagcatgtgtgttatgtgttgtgtgttggtggggcagattcttgcgagcactttggtctcagatggacctgctaccagttctctctgcagacccccataggtttctcctaaacctggcctctcctattaggcagccttactcagcggcagcttctcagctccatgttttcaaggaaccacaatttatttccagcatccactgaagcatattatcagtggtgatagagggggcttgtaaaactgtttttccacttaggtattagagggtggccattatttgagagtgactatgaccacagttaatctggtaataaattctcttgggtaggaggaaaggaaaggatgctttaaggaagcatcttgccaggagacacaaagctaacaagagtggagcctgcagctggagccgcagagcctaatcactacacccgcccatctctgctagggtttcatgacttcgtatcggggattagcagtatttaactctgttgcacaaacatttggtgtattattcaggtaacaagtagctaatagaggaagttttacttttttaagacataaatttgccttttcccaaattacttggtacatagtacttttcatgtttgaagttgagatgtgggtacaataccatagctttattccagagcagggtatttgtttccaaatgccatgttcccagcagctgcccttgactgggaattggggtgtgatttgggcttttccttaaatccttgaggagctggaggggtgggtggctcgcactcctgctttctggatctgaatcctgactctgtcatggacctgtttgactttgggcaagttgactcctattcctgagccccatatttttctcttctgtgaaattcagattaaaaaaacatggctttgatcaaacattataaataatatatagacagactgcttgtttttattgtattgccagaaatgaatcctactaatattgccatctatggacagaaaatgtattacctgtcttcatcaagacccagacgaggaagaacacgaaaagcggagattaattttactgccatctccagaaccgtcatcctaatatttacttacattttattattatttcaggctcatgcacatatacttagcatggatcattggccacagactcgcatacatttaactttattaccttttgcctcatgtatctcattaaaattttgctgcttaatcaaggatctgcatattattttaattttagaattcacagttccaagactttgaaagtttcaagcgttctgggtgaatgtgttatgctctctcccgccaccatgtctttataccccctgatttctcagccactatggcaaccactttctactcttagtagcccatatttagtccaatccccagctcaggagacacttcttccagggagccccctgtgccttccagtagtatcttgtacctgccctttttgcaaagctctttcctcctggcttagaatggcccattgacctgtttgtttctcctattaaactgtaagccactcgagggtagagagcatctgttgttcaccattgcatcctcggtgctgagcactgcgtctgacatattatttagaaggtcagtaagtgctagtgggattcaggctcccagtgggtgggagagaaaggacgtaaggaagcaagtggtaaaggccctcacagagtatcagcaggctggtgtgagggagaaatgcagaggatgggtgagtagcataatcgctaatgatagggtaatgatagagcacatttcacaacacctttaagccctttcacgtgcatcagataatttgatcctcataaaagcctagagatagatatattacagggatgaaggtggagtattttgtggttatgtgatatgtttaaaattatgcagtgagtaaatgactgggttcaaaccagaccttaaaagtctgttatctttccctcgagcatgcaatgaagtctacatcatccctaccatgtccatttgatcacaccctggcctcacagctctgtggtctacaggatacctcatggtggttttattgaccagacaataatcctctttctaaggggatgcatttcattaatacatatgtagatcatgaattgtctttgactttgaggggatggtagccagagcagaaagcaaagctgattttcatccccgtctggtaatgtggttggtaatgtgaagatgggtgtattctgagataccggctccttgcagtgtgtggttccttctgttttcaggcccaagaagcccatcctgggaaggaaaatgcattggggaaccctgtgcggattcttgtggctttggccctatcttttctatgtccaagctgtgcccatccaaaaagtccaagatgacaccaaaaccctcatcaagacaattgtcaccaggatcaatgacatttcacacacggtaaggagagtatgcggggacaaagtagaactgcagccagcccagcactggctcctagtggcactggacccagatagtccaagaaacatttattgaacgcctcctgaatgccaggcacctactggaagctgagaaggatttgaaagcacagggctccactctttctggttgtttcttttggcccctctgcctgctgagattccaggggttagtggttctaattctaaaccactccaagaacatttgattttgctacatgtttccatttaaaaatcataggatttgggctgggtgtggtggcttgtacctgtcatcccagcactttgggaggccaaagcaggaggatcattcgagcccaagagttcgagaccagcctgggcagcatagggagaccccatctctacaaaaataataaaaaatgttagctgggcatggtggtgtgtacctgtggtcccagctaggggaggctgagatggaaggatcacctgagcctgggaggttgaggctgcagtgggccctgatcatgccaccgtgctccagcctgggtgacagagtgagaccttgtctcaaaataaataaataaataaataaaagtcataggatttgatcaggcatgatgggtcacatctgtaagcccattgctttaggaggccaaggtaggaggatcagttgaggccaggagttcaagaccagcctgggcaacatggcaagacctctctctctaatttttaaaaaaataaaaattaaagataagaaaaaaatcataggattctcatgaggcctcacgtgcttattttcaacctaccaaggggaaacccaggcctcagcgattagctgagccacatgcaggcacagccactgtctctttccttcctgtcccctctgtccccaccttctgcgctcgccttcctccctgacttcacttccttgaatcttagtgcctacgaccagagggagctgtgaagttccttgtgtcccattggcaggaacaagacccccagaagcatctcctcagggcctctatcccatctctagatgtgcttgtcattagggttcttgtagttccagctgatctctggccctgccgctcaaagatacccaaaagagcgagtctaccctttttcacattcaaccctctactgatttgcaaatagcagtcagtgcccaccctggtcttttctctggggtccagcaggcctagaccttcagccattttcctgatgaggtctgtatttgaaattaggaagattaagtttgaatcttcacacttctgatgtctgtgagatcttcagcaagttccttactgtctttaagccttgttttcatcatctggataatggggatatcacacactattcacaaggttgttatgaggcctaaattagctaaagcaattgaatcctccttaccccctgcatggagctctctggagacttccacgtctcctggtcattgtgggtgtcttatggtagtcttgggcagttagggagaagttaggtgtctggaagcaaagatggctcagaactagatagagtcttgggcattttatagataaaaactcttgtctcctttaaaaataataaaaaaaaattagctgggcatattagccactcagcaagactgcacgtgatagatcccgagtgccccaccttgggtggtgtaatacacaatatcacgggagccccgggtagtaaccacggaggtgtcagcctcagtgctgtgggcagatggatggggagagcctcccggaactggagtcactggagcagggttggggggcctcactgagggtacggccttgatctctaaggaggagggactgcctggaaaagctgactgggagggaggactcggctgggggtagaagggactagggaaggctgggggtgggggtgcttatggaggacctcagatgcctggggaacagactccactaaataaaacatatgaaaccatggctggttcttcagcagaggccatgtagagaaaggaatgacctaggaaagttggcctggaagtggagggaaggatggtgtgggaaaagcaggaatctcggagaccagcttagaggcttggcagtcacctgggtgcaggatacaagggcctgagccaaagtggtgagggagggtggaaggaggcagcccagagaatgaccctccatgcccacggggaaggcagagggctctgagagcgattcctcccacatgctgagcacttgttctccctcttcctcctgcatagcagtcagtctcctccaaacagaaagtcaccggtttggacttcattcctgggctccaccccatcctgaccttatccaagatggaccagacactggcagtctaccaacagatcctcaccagtatgccttccagaaacgtgatccaaatatccaacgacctggagaacctccgggatcttcttcacgtgctggccttctctaagagctgccacttgccctgggccagtggcctggagaccttggacagcctggggggtgtcctggaagcttcaggctactccacagaggtggtggccctgagcaggctgcaggggtctctgcaggacatgctgtggcagctggacctcagccctgggtgctgaggccttgaaggtcactcttcctgcaaggactacgttaagggaaggaactctggcttccaggtatctccaggattgaagagcattgcatggacaccccttatccaggactctgtcaatttccctgactcctctaagccactcttccaaaggcataagaccctaagcctccttttgcttgaaaccaaagatatatacacaggatcctattctcaccaggaagggggtccacccagcaaagagtgggctgcatctgggattcccaccaaggtcttcagccatcaacaagagttgtcttgtcccctcttgacccatctccccctcactgaatgcctcaatgtgaccaggggtgatttcagagagggcagaggggtaggcagagcctttggatgaccagaacaaggttccctctgagaattccaaggagttccatgaagaccacatccacacacgcaggaactcccagcaacacaagctggaagcacatgtttatttattctgcattttattctggatggatttgaagcaaagcaccagcttctccaggctctttggggtcagccagggccaggggtctccctggagtgcagtttccaatcccatagatgggtctggctgagctgaacccattttgagtgactcgagggttgggttcatctgagcaagagctggcaaaggtggctctccagttagttctctcgtaactggtttcatttctactgtgactgatgttacatcacagtgtttgcaatggtgttgccctgagtggatctccaaggaccaggttattttaaaaagatttgttttgtcaagtgtcatatgtaggtgtctgcacccaggggtggggaatgtttgggcagaagggagaaggatctagaatgtgttttctgaataacatttgtgtggtgggttctttggaaggagtgagatcattttcttatcttctgcaattgcttaggatgtttttcatgaaaatagctctttcaggggggttgtgaggcctggccaggcaccccctggagagaagtttctggccctggctgaccccaaagagcctggagaagctgatgctttgcttcaaatccatccagaataaaacgcaaagggctgaaagccatttgttggggcagtggtaagctctggctttctccgactgctagggagtggtctttcctatcatggagtgacggtcccacactggtgactgcgatcttcagagcaggggtccttggtgtgaccctctgaatggtccagggttgatcacactctgggtttattacatggcagtgttcctatttggggcttgcatgccaaattgtagttcttgtctgattggctcacccaagcaaggccaaaattaccaaaaatcttggggggtttttactccagtggtgaagaaaactcctttagcaggtggtcctgagacctgacaagcactgctaggcgagtgccaggactccccaggccaggccaccaggatggcccttcccactggaggtcacattcaggaagatgaaagaggaggtttggggtctgccaccatcctgctgctgtgtttttgctatcacacagtgggtggtggatctgtccaaggaaacttgaatcaaagcagttaactttaagactgagcacctgcttcatgctcagccctgactggtgctataggctggagaagctcacccaataaacattaagattgaggcctgccctcagggatcttgcattcccagtggtcaaaccgcactcacccatgtgccaaggtggggtatttaccacagcagctgaacagccaaatgcatggtgcagttgacagcaggtgggaaatggtatgagctgaggggggccgtgcccaggggcccacagggaaccctgcttgcactttgtaacatgtttacttttcagggcatcttagcttctattatagccacatccctttgaaacaagataactgagaatttaaaaataagaaaatacataagaccataacagccaacaggtggcaggaccaggactatagcccaggtcctctgatacccagagcattacgtgagccaggtaatgagggactggaaccagggagaccgagcgctttctggaaaagaggagtttcgaggtagagtttgaaggaggtgagggatgtgaattgcctgcagagagaagcctgttttgttggaaggtttggtgtgtggagatgcagaggtaaaagtgtgagcagtgagttacagcgagaggcagagaaagaagagacaggagggcaagggccatgctgaagggaccttgaagggtaaagaagtttgatattaaaggagttaagagtagcaagttctagagaagaggctggtgctgtggccagggtgagagctgctctggaaaatgtgacccagatcctcacaaccacctaatcaggctgaggtgtcttaagccttttgctcacaaaacctggcacaatggctaattcccagagtgtgaaacttcctaagtataaatggttgtctgtttttgtaacttaaaaaaaaaaaaaaaagtttggccgggtgcggtggctcacgcctgtaatcccagcactttgggaggccaaggtggggggatcacaaggtcactagatggcgagcatcctggccaacatggtgaaaccccgtctctactaaaaacacaaaagttagctgagcgtggtggcgggcgcctgtagtcccagccactcgggaggctgagacaggagaatcgcttaaacctgggaggcggagagtacagtgagccaagatcgcgccactgcactccggcctgatgacagagcgagattccgtcttaaaaaaaaaaaaaaaaaagtttgtttttaaaaaaatctaaataaaataactttgccccctgc

SEQ ID NO: 15 - DNA, 89 bp, Homo sapiens
  source 1..89: mol_type = other DNA
tgctgctggccagagctcttttcacattgtgctactgtctgcacctgtcactagcagtgcaatgttaaaagggcattggccgtgtagtg

SEQ ID NO: 16 - DNA, 86 bp, Homo sapiens
  source 1..86: mol_type = other DNA
tggggccctggctgggatatcatcatatactgtaagtttgcgatgagacactacagtatagatgatgtactagtccgggcaccccc

SEQ ID NO: 17 - DNA, 87 bp, Homo sapiens
  source 1..87: mol_type = other DNA
cactgttctatggttagttttgcaggtttgcatccagctgtgtgatattctgctgtgcaaatccatgcaaaactgactgtggtagtg

SEQ ID NO: 18 - DNA, 69 bp, Homo sapiens
  source 1..69: mol_type = other DNA
ctgtggtgcattgtagttgcattgcatgttctggtggtacccatgcaatgtttccacagtgcatcacag